European Patent Application EP 4 410 836 A1, published August 7, 2024. Title: 联合治疗血液肿瘤的抗CD47抗体. Applicant: 正大天晴药业集团南京顺欣制药有限公司. Application CN. The sequence listing filed with the application follows.

SEQUENCE LISTING (198 sequences)

SEQ ID NO: 1 - protein, 10 aa, Mus musculus
GFSLTNYGVH

SEQ ID NO: 2 - protein, 10 aa, Mus musculus
GFTFSNYYMS

SEQ ID NO: 3 - protein, 10 aa, Mus musculus
GYTFTNYGMN

SEQ ID NO: 4 - protein, 10 aa, Mus musculus
GYTFSRYWIE

SEQ ID NO: 5 - protein, 10 aa, Mus musculus
GFNIEDDYIE

SEQ ID NO: 6 - protein, 9 aa, Mus musculus
IIWAGGSTN

SEQ ID NO: 7 - protein, 10 aa, Mus musculus
YISSGGGSTY

SEQ ID NO: 8 - protein, 10 aa, Mus musculus
WINTNTGEPT

SEQ ID NO: 9 - protein, 8 aa, Mus musculus
EFIPGSDT

SEQ ID NO: 10 - protein, 10 aa, Mus musculus
RIDPANDKTK

SEQ ID NO: 11 - protein, 8 aa, Mus musculus
DDYASMDY

SEQ ID NO: 12 - skipped

SEQ ID NO: 13 - protein, 10 aa, Mus musculus
FSHLRGPMDY

SEQ ID NO: 14 - protein, 8 aa, Mus musculus
GGLRRMDY

SEQ ID NO: 15 - protein, 11 aa, Mus musculus
PGLRRYYSMDY

SEQ ID NO: 16 - protein, 16 aa, Mus musculus
RSSQSLVHSNGNTYLH

SEQ ID NO: 17 - protein, 16 aa, Mus musculus
KSSQSLLDSDGKTYLN

SEQ ID NO: 18 - protein, 16 aa, Mus musculus
RSSQSLVHSNGYTYLH

SEQ ID NO: 19 - protein, 12 aa, Mus musculus
RASSSVSSTYLH

SEQ ID NO: 20 - protein, 11 aa, Mus musculus
KASENVVSYVS

SEQ ID NO: 21 - protein, 7 aa, Mus musculus
KVSNRFS

SEQ ID NO: 22 - protein, 7 aa, Mus musculus
LVSKLDS

SEQ ID NO: 23 - protein, 7 aa, Mus musculus
KVSNRFS

SEQ ID NO: 24 - protein, 7 aa, Mus musculus
TTSTLAS

SEQ ID NO: 25 - protein, 7 aa, Mus musculus
GASNRYT

SEQ ID NO: 26 - protein, 9 aa, Mus musculus
SQSTHVPYT

SEQ ID NO: 27 - protein, 7 aa, Mus musculus
GTHFPLT

SEQ ID NO: 28 - protein, 9 aa, Mus musculus
SQSTHVPPT

SEQ ID NO: 29 - protein, 9 aa, Mus musculus
QQFSDSTWT

SEQ ID NO: 30 - protein, 9 aa, Mus musculus
GQSYSYPLT

SEQ ID NO: 31 - protein, 9 aa, synthetic construct
  REGION 1..9: note = Light chain CDR3; note (original language) = 轻链互补决定区3
QQFSESTWT

SEQ ID NO: 32 - protein, 9 aa, synthetic construct
  MUTAGEN 5: note = X is D or E
  REGION 1..9: note = Light chain CDR3; note (original language) = 轻链互补决定区3
QQFSXSTWT

SEQ ID NO: 33 - protein, 116 aa, Mus musculus
QVQLKESGPGLVAPSQSLSITCTVSGFSLTNYGVHWVRQPPGKGLEWLGIIWAGGSTNYNSALMSRLSISKDNSKSQVFLKMNSLQTDDTAMYYCARDDYASMDYWGQGTSVTVSS

SEQ ID NO: 34 - protein, 112 aa, Mus musculus
DAFMTQTPLSLPVSLGDQASISCRSSQSLVHSNGNTYLHWYLQKPGQSPKLLIYKVSNRFSGVPDRFSGSGSGTDFTLKISRVEAEDLGVYFCSQSTHVPYTLGGGTKLEIK

SEQ ID NO: 35 - protein, 119 aa, Mus musculus
EVQLQQSGPELKKPGETVKISCKASGYTFTNYGMNWVKQVPGKGLKWMGWINTNTGEPTYAEEFKGRFAFSLETSARTAFLQINNLKNEDTATYFCTRFSHLRGPMDYWGQGASVTVSS

SEQ ID NO: 36 - protein, 112 aa, Mus musculus
DAVMTQTPLSLPVSLGDQASISCRSSQSLVHSNGYTYLHWYLQKPGQSPKLLIYKVSNRFSGVPDRFSGSGSGTDFTLKISRLEAEDLGVYFCSQSTHVPPTFGGGTKLEIK

SEQ ID NO: 37 - protein, 112 aa, Mus musculus
EVMLVESGGGLVQPGGSLKLSCAASGFTFSNYYMSWVRQTPEKRLEWVAYISSGGGSTYYPDSVKGRFTISRDNAKNTLYLQMSSLKSEDTAMYYCAWFAYWGQGTLVTVSA

SEQ ID NO: 38 - protein, 112 aa, Mus musculus
DAVVTQTPLTLSVTIGQPASISCKSSQSLLDSDGKTYLNWLLQRPGQSPKRLIYLVSKLDSGVPDRFTGSGSGTDFTLKISRVEAEDLGVYYCWQGTHFPLTFGAGTKLELK

SEQ ID NO: 39 - protein, 117 aa, Mus musculus
EVQLQQSVAELMKPGASVKIYCKATGYTFSRYWIEWVKQRPGHGLEWIGEFIPGSDTTNFNEKFKGKATFTAEISSNTAYMQLSSLTSEDSAVYFCARGGLRRMDYWGQGTSVTVSS

SEQ ID NO: 40 - protein, 108 aa, Mus musculus
DIVMTQTPAIMSASPGEKVTMTCRASSSVSSTYLHWYQQKSGASPKLWIYTTSTLASGVPARFSGSGSGTSYSLTISSVEAEDAATYYCQQFSDSTWTFGGGTKLEIK

SEQ ID NO: 41 - protein, 120 aa, Mus musculus
EVQLQQSGAEVARPGASVKLSCTVSGFNIEDDYIEWVKQRPEQGLEWIGRIDPANDKTKYAPKFQDKATITGDTSSNTAYLQLSSLTSEDTAVYYCTRPGLRRYYSMDYWGQGTSVTVSS

SEQ ID NO: 42 - protein, 107 aa, Mus musculus
NIVLTQSPKSMSMSVGERVTLSCKASENVVSYVSWYQQKPEQSPKLLIYGASNRYTGVPDRFIGSGSSTDFTLIISSFQPEDLADYHCGQSYSYPLTFGAGTKLELK

SEQ ID NO: 43 - protein, 117 aa, synthetic construct
  REGION 1..117: note = VH; note (original language) = 重链可变区
QVQLVQSGAEVKKPGSSVKVSCKASGYTFSRYWIEWVRQAPGQGLEWMGEFIPGSDTTNYAQKFQGRVTITADISTSTAYMELSSLRSEDTAVYYCARGGLRRMDYWGQGTLVTVSS

SEQ ID NO: 44 - protein, 108 aa, synthetic construct
  REGION 1..108: note = VL; note (original language) = 轻链可变区
DIQMTQSPSSLSASVGDRVTITCRASSSVSSTYLHWYQQKPGKAPKLLIYTTSTLASGVPSRFSGSGSGTDFTLTISSLQPEDFATYYCQQFSDSTWTFGQGTKLEIK

SEQ ID NO: 45 - protein, 117 aa, synthetic construct; identical to SEQ ID NO: 43
  REGION 1..117: note = VH; note (original language) = 重链可变区

SEQ ID NO: 46 - protein, 108 aa, synthetic construct
  REGION 1..108: note = VL; note (original language) = 轻链可变区
DIQMTQSPSSLSASVGDRVTITCRASSSVSSTYLHWYQQKPGKAPKLLIYTTSTLASGVPSRFSGSGSGTDFTLTISSLQPEDFATYYCQQFSESTWTFGQGTKLEIK

SEQ ID NO: 47 - protein, 117 aa, synthetic construct; identical to SEQ ID NO: 43
  REGION 1..117: note = VH; note (original language) = 重链可变区

SEQ ID NO: 48 - protein, 108 aa, synthetic construct
  REGION 1..108: note = VL; note (original language) = 轻链可变区
DIQMTQSPSSLSASVGDRVTITCRASSSVSSTYLHWYQQKPGKAPKLLIYTTSTLASGVPSRFSGSGSGTSYTLTISSLQPEDFATYYCQQFSDSTWTFGQGTKLEIK

SEQ ID NO: 49 - protein, 117 aa, synthetic construct; identical to SEQ ID NO: 43
  REGION 1..117: note = VH; note (original language) = 重链可变区

SEQ ID NO: 50 - protein, 108 aa, synthetic construct
  REGION 1..108: note = VL; note (original language) = 轻链可变区
DIQMTQSPSSLSASVGDRVTITCRASSSVSSTYLHWYQQKPGKAPKLLIYTTSTLASGVPSRFSGSGSGTSYTLTISSLQPEDFATYYCQQFSESTWTFGQGTKLEIK

SEQ ID NO: 51 - protein, 117 aa, synthetic construct; identical to SEQ ID NO: 43
  REGION 1..117: note = VH; note (original language) = 重链可变区

SEQ ID NO: 52 - protein, 108 aa, synthetic construct
  REGION 1..108: note = VL; note (original language) = 轻链可变区
DIQMTQSPSSLSASVGDRVTITCRASSSVSSTYLHWYQQKPGKAPKLWIYTTSTLASGVPSRFSGSGSGTSYTLTISSLQPEDFATYYCQQFSDSTWTFGQGTKLEIK

SEQ ID NO: 53 - protein, 117 aa, synthetic construct; identical to SEQ ID NO: 43
  REGION 1..117: note = VH; note (original language) = 重链可变区

SEQ ID NO: 54 - protein, 108 aa, synthetic construct
  REGION 1..108: note = VL; note (original language) = 轻链可变区
DIQMTQSPSSLSASVGDRVTITCRASSSVSSTYLHWYQQKPGKAPKLWIYTTSTLASGVPSRFSGSGSGTSYTLTISSLQPEDFATYYCQQFSESTWTFGQGTKLEIK

SEQ ID NO: 55 - protein, 117 aa, synthetic construct
  REGION 1..117: note = VH; note (original language) = 重链可变区
QVQLVQSGAEVKKPGSSVKVSCKASGYTFSRYWIEWVRQAPGQGLEWMGEFIPGSDTTNYAQKFQGRVTITAEISTNTAYMELSSLRSEDTAVYYCARGGLRRMDYWGQGTLVTVSS

SEQ ID NO: 56 - protein, 108 aa, synthetic construct; identical to SEQ ID NO: 44
  REGION 1..108: note = VL; note (original language) = 轻链可变区

SEQ ID NO: 57 - protein, 117 aa, synthetic construct; identical to SEQ ID NO: 55
  REGION 1..117: note = VH; note (original language) = 重链可变区

SEQ ID NO: 58 - protein, 108 aa, synthetic construct; identical to SEQ ID NO: 46
  REGION 1..108: note = VL; note (original language) = 轻链可变区

SEQ ID NO: 59 - protein, 117 aa, synthetic construct; identical to SEQ ID NO: 55
  REGION 1..117: note = VH; note (original language) = 重链可变区

SEQ ID NO: 60 - protein, 108 aa, synthetic construct; identical to SEQ ID NO: 48
  REGION 1..108: note = VL; note (original language) = 轻链可变区

SEQ ID NO: 61 - protein, 117 aa, synthetic construct; identical to SEQ ID NO: 55
  REGION 1..117: note = VH; note (original language) = 重链可变区

SEQ ID NO: 62 - protein, 108 aa, synthetic construct; identical to SEQ ID NO: 50
  REGION 1..108: note = VL; note (original language) = 轻链可变区

SEQ ID NO: 63 - protein, 117 aa, synthetic construct; identical to SEQ ID NO: 55
  REGION 1..117: note = VH; note (original language) = 重链可变区

SEQ ID NO: 64 - protein, 108 aa, synthetic construct; identical to SEQ ID NO: 52
  REGION 1..108: note = VL; note (original language) = 轻链可变区

SEQ ID NO: 65 - protein, 117 aa, synthetic construct; identical to SEQ ID NO: 55
  REGION 1..117: note = VH; note (original language) = 重链可变区

SEQ ID NO: 66 - protein, 108 aa, synthetic construct; identical to SEQ ID NO: 54
  REGION 1..108: note = VL; note (original language) = 轻链可变区

SEQ ID NO: 67 - protein, 119 aa, synthetic construct
  REGION 1..119: note = VH; note (original language) = 重链可变区
QVQLVQSGAEVKKPGASVKVSCKASGYTFTNYGMNWVRQAPGQGLEWMGWINTNTGEPTYAQKLQGRVTMTLDTSTRTAYMELRSLRSDDTAVYYCARFSHLRGPMDYWGQGTLVTVSS

SEQ ID NO: 68 - protein, 112 aa, synthetic construct
  REGION 1..112: note = VL; note (original language) = 轻链可变区
DIQMTQSPSSLSASVGDRVTITCRSSQSLVHSNGYTYLHWYQQKPGKAPKLLIYKVSNRFSGVPSRFSGSGSGTDFTLTISSLQPEDFATYYCSQSTHVPPTFGQGTKLEIK

SEQ ID NO: 69 - protein, 119 aa, synthetic construct
  REGION 1..119: note = VH; note (original language) = 重链可变区
QVQLVQSGAEVKKPGASVKVSCKASGYTFTNYGMNWVRQAPGQGLKWMGWINTNTGEPTYAQELQGRVTMTLDTSTRTAYMELRSLRSDDTAVYYCTRFSHLRGPMDYWGQGTLVTVSS

SEQ ID NO: 70 - protein, 112 aa, synthetic construct; identical to SEQ ID NO: 68
  REGION 1..112: note = VL; note (original language) = 轻链可变区

SEQ ID NO: 71 - protein, 119 aa, synthetic construct
  REGION 1..119: note = VH; note (original language) = 重链可变区
QVQLVQSGAEVKKPGASVKVSCKASGYTFTNYGMNWVRQAPGQGLKWMGWINTNTGEPTYAQELQGRVTMTLDTSTRTAYMELRSLRSDDTAVYYCARFSHLRGPMDYWGQGTLVTVSS

SEQ ID NO: 72 - protein, 112 aa, synthetic construct; identical to SEQ ID NO: 68
  REGION 1..112: note = VL; note (original language) = 轻链可变区

SEQ ID NO: 73 - protein, 119 aa, synthetic construct; identical to SEQ ID NO: 71
  REGION 1..119: note = VH; note (original language) = 重链可变区

SEQ ID NO: 74 - protein, 112 aa, synthetic construct
  REGION 1..112: note = VL; note (original language) = 轻链可变区
DAQMTQSPSSLSASVGDRVTITCRSSQSLVHSNGYTYLHWYQQKPGKAPKLLIYKVSNRFSGVPSRFSGSGSGTDFTLTISSLQPEDFATYYCSQSTHVPPTFGQGTKLEIK

SEQ ID NO: 75 - protein, 119 aa, synthetic construct; identical to SEQ ID NO: 67
  REGION 1..119: note = VH; note (original language) = 重链可变区

SEQ ID NO: 76 - protein, 112 aa, synthetic construct; identical to SEQ ID NO: 74
  REGION 1..112: note = VL; note (original language) = 轻链可变区

SEQ ID NO: 77 - protein, 119 aa, synthetic construct; identical to SEQ ID NO: 69
  REGION 1..119: note = VH; note (original language) = 重链可变区

SEQ ID NO: 78 - protein, 112 aa, synthetic construct; identical to SEQ ID NO: 74
  REGION 1..112: note = VL; note (original language) = 轻链可变区

SEQ ID NO: 79 - protein, 120 aa, synthetic construct
  REGION 1..120: note = VH; note (original language) = 重链可变区
QVQLVQSGAEVKKPGASVKVSCKVSGFNIEDDYIEWVRQAPGQGLEWMGRIDPANDKTKYAQKFQGRVTMTGDTSTNTVYMELSSLRSEDTAVYYCARPGLRRYYSMDYWGQGTLVTVSS

SEQ ID NO: 80 - protein, 107 aa, synthetic construct
  REGION 1..107: note = VL; note (original language) = 轻链可变区
DIQMTQSPSSLSASVGDRVTITCKASENVVSYVSWYQQKPGKAPKLLIYGASNRYTGVPSRFIGSGSSTDFTLTISSLQPEDFATYYCGQSYSYPLTFGQGTKLEIK

SEQ ID NO: 81 - protein, 120 aa, synthetic construct
  REGION 1..120: note = VH; note (original language) = 重链可变区
QVQLVQSGAEVKKPGASVKVSCKVSGFNIEDDYIEWVRQAPGQGLEWMGRIDPANDKTKYAQKFQGRVTMTGDTSTNTVYMELSSLRSEDTAVYYCTRPGLRRYYSMDYWGQGTLVTVSS

SEQ ID NO: 82 - protein, 107 aa, synthetic construct; identical to SEQ ID NO: 80
  REGION 1..107: note = VL; note (original language) = 轻链可变区

SEQ ID NO: 83 - protein, 117 aa, synthetic construct
  MUTAGEN 73: note = X is D or E
  MUTAGEN 74: note = X is I or E
  MUTAGEN 77: note = X is S or N
  REGION 1..117: note = VH; note (original language) = 重链可变区
QVQLVQSGAEVKKPGSSVKVSCKASGYTFSRYWIEWVRQAPGQGLEWMGEFIPGSDTTNYAQKFQGRVTITAXXSTXTAYMELSSLRSEDTAVYYCARGGLRRMDYWGQGTLVTVSS

SEQ ID NO: 84 - protein, 108 aa, synthetic construct
  MUTAGEN 48: note = X is L or W
  MUTAGEN 71: note = X is D or S
  MUTAGEN 72: note = X is F or Y
  MUTAGEN 94: note = X is D or E
  REGION 1..108: note = VL; note (original language) = 轻链可变区
DIQMTQSPSSLSASVGDRVTITCRASSSVSSTYLHWYQQKPGKAPKLXIYTTSTLASGVPSRFSGSGSGTXXTLTISSLQPEDFATYYCQQFSXSTWTFGQGTKLEIK

SEQ ID NO: 85 - protein, 119 aa, synthetic construct
  MUTAGEN 46: note = X is E or K
  MUTAGEN 63: note = X is E or K
  MUTAGEN 72: note = X is L or T
  MUTAGEN 77: note = X is R or S
  MUTAGEN 97: note = X is A or T
  REGION 1..119: note = VH; note (original language) = 重链可变区
QVQLVQSGAEVKKPGASVKVSCKASGYTFTNYGMNWVRQAPGQGLXWMGWINTNTGEPTYAQXLQGRVTMTXDTSTXTAYMELRSLRSDDTAVYYCXRFSHLRGPMDYWGQGTLVTVSS

SEQ ID NO: 86 - protein, 112 aa, synthetic construct
  MUTAGEN 2: note = X is I or A
  REGION 1..112: note = VL; note (original language) = 轻链可变区
DXQMTQSPSSLSASVGDRVTITCRSSQSLVHSNGYTYLHWYQQKPGKAPKLLIYKVSNRFSGVPSRFSGSGSGTDFTLTISSLQPEDFATYYCSQSTHVPPTFGQGTKLEIK

SEQ ID NO: 87 - protein, 120 aa, synthetic construct
  MUTAGEN 24: note = X is A or V
  MUTAGEN 72: note = X is R or G
  MUTAGEN 97: note = X is A or T
  MUTAGEN 77: note = X is S or N
  REGION 1..120: note = VH; note (original language) = 重链可变区
QVQLVQSGAEVKKPGASVKVSCKXSGFNIEDDYIEWVRQAPGQGLEWMGRIDPANDKTKYAQKFQGRVTMTXDTSTXTVYMELSSLRSEDTAVYYCXRPGLRRYYSMDYWGQGTLVTVSS

SEQ ID NO: 88 - protein, 107 aa, synthetic construct
  MUTAGEN 63: note = X is S or I
  MUTAGEN 68: note = X is S or G
  REGION 1..107: note = VL; note (original language) = 轻链可变区
DIQMTQSPSSLSASVGDRVTITCKASENVVSYVSWYQQKPGKAPKLLIYGASNRYTGVPSRFXGSGSXTDFTLTISSLQPEDFATYYCGQSYSYPLTFGQGTKLEIK

SEQ ID NO: 89 - protein, 443 aa, synthetic construct
  REGION 1..443: note = Heavy chain; note (original language) = 重链
QVQLKESGPGLVAPSQSLSITCTVSGFSLTNYGVHWVRQPPGKGLEWLGIIWAGGSTNYNSALMSRLSISKDNSKSQVFLKMNSLQTDDTAMYYCARDDYASMDYWGQGTSVTVSSASTKGPSVFPLAPCSRSTSESTAALGCLVKDYFPEPVTVSWNSGALTSGVHTFPAVLQSSGLYSLSSVVTVPSSSLGTKTYTCNVDHKPSNTKVDKRVESKYGPPCPPCPAPEFLGGPSVFLFPPKPKDTLMISRTPEVTCVVVDVSQEDPEVQFNWYVDGVEVHNAKTKPREEQFNSTYRVVSVLTVLHQDWLNGKEYKCKVSNKGLPSSIEKTISKAKGQPREPQVYTLPPSQEEMTKNQVSLTCLVKGFYPSDIAVEWESNGQPENNYKTTPPVLDSDGSFFLYSRLTVDKSRWQEGNVFSCSVMHEALHNHYTQKSLSLSLGK

SEQ ID NO: 90 - DNA, 1332 bp, synthetic construct
  source 1..1332: mol_type = other DNA
  gene 1..1332: note = Nucleic acid encoding chimeric heavy chain; note (original language) = 重链编码核酸
caggtgcagctgaaggagtctggaccaggactggtggctccatctcagtccctgagcatcacctgcacagtgtccggcttcagcctgaccaactacggagtgcactgggtgaggcagccacctggcaagggactggagtggctgggcatcatctgggctggcggctccacaaactataattctgccctgatgtcccggctgtctatctccaaggacaacagcaagtctcaggtgtttctgaagatgaatagcctgcagaccgacgatacagccatgtactattgtgctagggacgattacgccagcatggattattggggccagggcacctctgtgacagtgtccagcgcctctacaaagggcccttccgtgttcccactggctccctgctccagaagcacatctgagtccaccgccgctctgggctgtctggtgaaggactacttccctgagccagtgaccgtgtcctggaacagcggcgccctgacatctggcgtgcacacctttccagctgtgctgcagtccagcggcctgtactccctgtcttccgtggtgacagtgcccagctcttccctgggcaccaagacatatacctgcaacgtggaccataagccttccaataccaaggtggataagagggtggagagcaagtacggaccaccttgcccaccatgtccagctcctgagtttctgggaggaccatccgtgttcctgtttcctccaaagcctaaggacaccctgatgatcagccggacacctgaggtgacctgcgtggtggtggacgtgtctcaggaggatccagaggtgcagttcaactggtacgtggatggcgtggaggtgcacaatgctaagaccaagccaagagaggagcagtttaattccacataccgcgtggtgagcgtgctgaccgtgctgcatcaggattggctgaacggcaaggagtataagtgcaaggtgtccaataagggcctgcccagctctatcgagaagacaatcagcaaggctaagggacagcctagggagccacaggtgtacaccctgcccccttctcaggaggagatgacaaagaaccaggtgtccctgacctgtctggtgaagggcttctatccaagcgacatcgctgtggagtgggagtctaatggccagcccgagaacaattacaagaccacaccacccgtgctggactctgatggctccttctttctgtattctaggctgacagtggataagtcccggtggcaggagggcaacgtgtttagctgctctgtgatgcacgaggccctgcacaatcattatacccagaagtccctgagcctgtctctgggcaagtga

SEQ ID NO: 91 - protein, 219 aa, synthetic construct
  REGION 1..219: note = Light chain; note (original language) = 轻链
DAFMTQTPLSLPVSLGDQASISCRSSQSLVHSNGNTYLHWYLQKPGQSPKLLIYKVSNRFSGVPDRFSGSGSGTDFTLKISRVEAEDLGVYFCSQSTHVPYTLGGGTKLEIKRTVAAPSVFIFPPSDEQLKSGTASVVCLLNNFYPREAKVQWKVDNALQSGNSQESVTEQDSKDSTYSLSSTLTLSKADYEKHKVYACEVTHQGLSSPVTKSFNRGEC

SEQ ID NO: 92 - DNA, 660 bp, synthetic construct
  source 1..660: mol_type = other DNA
  gene 1..660: note = Nucleic acid encoding chimeric light chain; note (original language) = 轻链编码核酸
gacgccttcatgacccagacaccactgtccctgcctgtgagcctgggcgatcaggcttctatctcctgcagatccagccagtctctggtgcactccaacggcaatacatacctgcattggtatctgcagaagccaggccagtcccccaagctgctgatctacaaggtgagcaacaggttctctggcgtgcctgaccggtttagcggctctggctccggcaccgatttcacactgaagatctccagggtggaggctgaggacctgggcgtgtacttttgtagccagtctacccacgtgccatatacactgggcggcggcaccaagctggagatcaagcgtacggtggccgctcccagcgtgttcatctttcccccttctgacgagcagctgaagtctggcaccgcttccgtggtgtgcctgctgaacaatttctaccccagagaggccaaggtgcagtggaaggtggataacgctctgcagtccggcaatagccaggagtctgtgaccgagcaggactccaaggatagcacatattctctgtcttccaccctgacactgtctaaggccgactacgagaagcacaaggtgtatgcttgcgaggtgacccatcagggcctgagctctcctgtgacaaagtcctttaatcgcggcgagtgttga

SEQ ID NO: 93 - protein, 446 aa, synthetic construct
  REGION 1..446: note = Heavy chain; note (original language) = 重链
EVQLQQSGPELKKPGETVKISCKASGYTFTNYGMNWVKQVPGKGLKWMGWINTNTGEPTYAEEFKGRFAFSLETSARTAFLQINNLKNEDTATYFCTRFSHLRGPMDYWGQGASVTVSSASTKGPSVFPLAPCSRSTSESTAALGCLVKDYFPEPVTVSWNSGALTSGVHTFPAVLQSSGLYSLSSVVTVPSSSLGTKTYTCNVDHKPSNTKVDKRVESKYGPPCPPCPAPEFLGGPSVFLFPPKPKDTLMISRTPEVTCVVVDVSQEDPEVQFNWYVDGVEVHNAKTKPREEQFNSTYRVVSVLTVLHQDWLNGKEYKCKVSNKGLPSSIEKTISKAKGQPREPQVYTLPPSQEEMTKNQVSLTCLVKGFYPSDIAVEWESNGQPENNYKTTPPVLDSDGSFFLYSRLTVDKSRWQEGNVFSCSVMHEALHNHYTQKSLSLSLGK

SEQ ID NO: 94 - DNA, 1341 bp, synthetic construct
  source 1..1341: mol_type = other DNA
  gene 1..1341: note = Nucleic acid encoding chimeric heavy chain; note (original language) = 重链编码核酸
gaggtgcagctgcagcagtctggccccgagctgaagaagcctggcgagaccgtgaagatctcttgcaaggcctccggctacaccttcacaaactatggcatgaattgggtgaagcaggtgccaggcaagggcctgaagtggatgggctggatcaacaccaatacaggcgagcccacatacgccgaggagttcaagggcagattcgcttttagcctggagacctctgcccgcacagcttttctgcagatcaacaatctgaagaacgaggacaccgccacatacttctgtaccaggttttcccacctgcggggccccatggattattggggccagggcgctagcgtgacagtgtccagcgcctctacaaagggcccttccgtgttcccactggctccctgctccagaagcacatctgagtccaccgccgctctgggctgtctggtgaaggactacttccctgagccagtgaccgtgtcctggaacagcggcgccctgacatctggcgtgcacacctttccagctgtgctgcagtccagcggcctgtactccctgtcttccgtggtgacagtgcccagctcttccctgggcaccaagacatatacctgcaacgtggaccataagccttccaataccaaggtggataagagggtggagagcaagtacggaccaccttgcccaccatgtccagctcctgagtttctgggaggaccatccgtgttcctgtttcctccaaagcctaaggacaccctgatgatcagccggacacctgaggtgacctgcgtggtggtggacgtgtctcaggaggatccagaggtgcagttcaactggtacgtggatggcgtggaggtgcacaatgctaagaccaagccaagagaggagcagtttaattccacataccgcgtggtgagcgtgctgaccgtgctgcatcaggattggctgaacggcaaggagtataagtgcaaggtgtccaataagggcctgcccagctctatcgagaagacaatcagcaaggctaagggacagcctagggagccacaggtgtacaccctgcccccttctcaggaggagatgacaaagaaccaggtgtccctgacctgtctggtgaagggcttctatccaagcgacatcgctgtggagtgggagtctaatggccagcccgagaacaattacaagaccacaccacccgtgctggactctgatggctccttctttctgtattctaggctgacagtggataagtcccggtggcaggagggcaacgtgtttagctgctctgtgatgcacgaggccctgcacaatcattatacccagaagtccctgagcctgtctctgggcaagtga

SEQ ID NO: 95 - protein, 219 aa, synthetic construct
  REGION 1..219: note = Light chain; note (original language) = 轻链
DAVMTQTPLSLPVSLGDQASISCRSSQSLVHSNGYTYLHWYLQKPGQSPKLLIYKVSNRFSGVPDRFSGSGSGTDFTLKISRLEAEDLGVYFCSQSTHVPPTFGGGTKLEIKRTVAAPSVFIFPPSDEQLKSGTASVVCLLNNFYPREAKVQWKVDNALQSGNSQESVTEQDSKDSTYSLSSTLTLSKADYEKHKVYACEVTHQGLSSPVTKSFNRGEC

SEQ ID NO: 96 - DNA, 660 bp, synthetic construct
  source 1..660: mol_type = other DNA
  gene 1..660: note = Nucleic acid encoding chimeric light chain; note (original language) = 轻链编码核酸
gacgccgtgatgacccagacaccactgtccctgcccgtgagcctgggcgatcaggcttctatctcctgcagatccagccagtctctggtgcactccaacggctacacatatctgcattggtacctgcagaagcctggccagtccccaaagctgctgatctataaggtgagcaataggttctctggagtgccagaccggtttagcggatctggatccggcaccgatttcacactgaagatctccaggctggaggctgaggacctgggcgtgtacttctgtagccagtctacccacgtgccccctacatttggcggcggcaccaagctggagatcaagcgtacggtggccgctcccagcgtgttcatctttcccccttctgacgagcagctgaagtctggcaccgcttccgtggtgtgcctgctgaacaatttctaccccagagaggccaaggtgcagtggaaggtggataacgctctgcagtccggcaatagccaggagtctgtgaccgagcaggactccaaggatagcacatattctctgtcttccaccctgacactgtctaaggccgactacgagaagcacaaggtgtatgcttgcgaggtgacccatcagggcctgagctctcctgtgacaaagtcctttaatcgcggcgagtgttga

SEQ ID NO: 97 - protein, 439 aa, synthetic construct
  REGION 1..439: note = Heavy chain; note (original language) = 重链
EVMLVESGGGLVQPGGSLKLSCAASGFTFSNYYMSWVRQTPEKRLEWVAYISSGGGSTYYPDSVKGRFTISRDNAKNTLYLQMSSLKSEDTAMYYCAWFAYWGQGTLVTVSAASTKGPSVFPLAPCSRSTSESTAALGCLVKDYFPEPVTVSWNSGALTSGVHTFPAVLQSSGLYSLSSVVTVPSSSLGTKTYTCNVDHKPSNTKVDKRVESKYGPPCPPCPAPEFLGGPSVFLFPPKPKDTLMISRTPEVTCVVVDVSQEDPEVQFNWYVDGVEVHNAKTKPREEQFNSTYRVVSVLTVLHQDWLNGKEYKCKVSNKGLPSSIEKTISKAKGQPREPQVYTLPPSQEEMTKNQVSLTCLVKGFYPSDIAVEWESNGQPENNYKTTPPVLDSDGSFFLYSRLTVDKSRWQEGNVFSCSVMHEALHNHYTQKSLSLSLGK

SEQ ID NO: 98 - DNA, 1320 bp, synthetic construct
  source 1..1320: mol_type = other DNA
  gene 1..1320: note = Nucleic acid encoding chimeric heavy chain; note (original language) = 重链编码核酸
gaagtgatgctggtggagagcggaggaggactggtgcagccaggaggcagcctgaagctgtcttgcgccgcttccggcttcacctttagcaactactatatgtcttgggtgagacagacacccgagaagcgcctggagtgggtggcttacatctccagcggaggaggatccacctactatcctgacagcgtgaagggcaggttcaccatctctcgggataacgccaagaatacactgtacctgcagatgtcttccctgaagtccgaggacacagctatgtactattgtgcctggtttgcttattggggccagggcaccctggtgacagtgtctgctgcctctacaaagggcccttccgtgttcccactggctccctgctccagaagcacatctgagtccaccgccgctctgggctgtctggtgaaggactacttccctgagccagtgaccgtgtcctggaacagcggcgccctgacatctggcgtgcacacctttccagctgtgctgcagtccagcggcctgtactccctgtcttccgtggtgacagtgcccagctcttccctgggcaccaagacatatacctgcaacgtggaccataagccttccaataccaaggtggataagagggtggagagcaagtacggaccaccttgcccaccatgtccagctcctgagtttctgggaggaccatccgtgttcctgtttcctccaaagcctaaggacaccctgatgatcagccggacacctgaggtgacctgcgtggtggtggacgtgtctcaggaggatccagaggtgcagttcaactggtacgtggatggcgtggaggtgcacaatgctaagaccaagccaagagaggagcagtttaattccacataccgcgtggtgagcgtgctgaccgtgctgcatcaggattggctgaacggcaaggagtataagtgcaaggtgtccaataagggcctgcccagctctatcgagaagacaatcagcaaggctaagggacagcctagggagccacaggtgtacaccctgcccccttctcaggaggagatgacaaagaaccaggtgtccctgacctgtctggtgaagggcttctatccaagcgacatcgctgtggagtgggagtctaatggccagcccgagaacaattacaagaccacaccacccgtgctggactctgatggctccttctttctgtattctaggctgacagtggataagtcccggtggcaggagggcaacgtgtttagctgctctgtgatgcacgaggccctgcacaatcattatacccagaagtccctgagcctgtctctgggcaagtga

SEQ ID NO: 99 - protein, 219 aa, synthetic construct
  REGION 1..219: note = Light chain; note (original language) = 轻链
DAVVTQTPLTLSVTIGQPASISCKSSQSLLDSDGKTYLNWLLQRPGQSPKRLIYLVSKLDSGVPDRFTGSGSGTDFTLKISRVEAEDLGVYYCWQGTHFPLTFGAGTKLELKRTVAAPSVFIFPPSDEQLKSGTASVVCLLNNFYPREAKVQWKVDNALQSGNSQESVTEQDSKDSTYSLSSTLTLSKADYEKHKVYACEVTHQGLSSPVTKSFNRGEC

SEQ ID NO: 100 - DNA, 660 bp, synthetic construct
  source 1..660: mol_type = other DNA
  gene 1..660: note = Nucleic acid encoding chimeric light chain; note (original language) = 轻链编码核酸
gacgccgtggtgacccagacaccactgaccctgtccgtgacaatcggccagcccgcttctatctcctgcaagtccagccagtccctgctggacagcgatggcaagacatacctgaactggctgctgcagaggccaggacagagccctaagcggctgatctatctggtgtctaagctggactccggcgtgcctgatagattcaccggcagcggctctggcaccgactttacactgaagatctctcgcgtggaggccgaggatctgggcgtgtactattgttggcagggcacccacttcccactgacatttggcgctggcaccaagctggagctgaagcgtacggtggccgctcccagcgtgttcatctttcccccttctgacgagcagctgaagtctggcaccgcttccgtggtgtgcctgctgaacaatttctaccccagagaggccaaggtgcagtggaaggtggataacgctctgcagtccggcaatagccaggagtctgtgaccgagcaggactccaaggatagcacatattctctgtcttccaccctgacactgtctaaggccgactacgagaagcacaaggtgtatgcttgcgaggtgacccatcagggcctgagctctcctgtgacaaagtcctttaatcgcggcgagtgttga

SEQ ID NO: 101 - protein, 444 aa, synthetic construct
  REGION 1..444: note = Heavy chain; note (original language) = 重链
EVQLQQSVAELMKPGASVKIYCKATGYTFSRYWIEWVKQRPGHGLEWIGEFIPGSDTTNFNEKFKGKATFTAEISSNTAYMQLSSLTSEDSAVYFCARGGLRRMDYWGQGTSVTVSSASTKGPSVFPLAPCSRSTSESTAALGCLVKDYFPEPVTVSWNSGALTSGVHTFPAVLQSSGLYSLSSVVTVPSSSLGTKTYTCNVDHKPSNTKVDKRVESKYGPPCPPCPAPEFLGGPSVFLFPPKPKDTLMISRTPEVTCVVVDVSQEDPEVQFNWYVDGVEVHNAKTKPREEQFNSTYRVVSVLTVLHQDWLNGKEYKCKVSNKGLPSSIEKTISKAKGQPREPQVYTLPPSQEEMTKNQVSLTCLVKGFYPSDIAVEWESNGQPENNYKTTPPVLDSDGSFFLYSRLTVDKSRWQEGNVFSCSVMHEALHNHYTQKSLSLSLGK

SEQ ID NO: 102 - DNA, 1335 bp, synthetic construct
  source 1..1335: mol_type = other DNA
  gene 1..1335: note = Nucleic acid encoding chimeric heavy chain; note (original language) = 重链编码核酸
gaggtgcagctgcagcagtctgtggccgagctgatgaagccaggcgcttccgtgaagatctactgcaaggccaccggctacacattcagcagatattggatcgagtgggtgaagcagaggccaggacacggactggagtggatcggcgagttcatccctggctctgacaccacaaacttcaatgagaagtttaagggcaaggccacctttacagctgagatctccagcaacaccgcttatatgcagctgtcttccctgacatccgaggacagcgccgtgtacttttgtgctaggggcggcctgaggcggatggattattggggccagggcacctccgtgacagtgagctctgcctctacaaagggcccttccgtgttcccactggctccctgctccagaagcacatctgagtccaccgccgctctgggctgtctggtgaaggactacttccctgagccagtgaccgtgtcctggaacagcggcgccctgacatctggcgtgcacacctttccagctgtgctgcagtccagcggcctgtactccctgtcttccgtggtgacagtgcccagctcttccctgggcaccaagacatatacctgcaacgtggaccataagccttccaataccaaggtggataagagggtggagagcaagtacggaccaccttgcccaccatgtccagctcctgagtttctgggaggaccatccgtgttcctgtttcctccaaagcctaaggacaccctgatgatcagccggacacctgaggtgacctgcgtggtggtggacgtgtctcaggaggatccagaggtgcagttcaactggtacgtggatggcgtggaggtgcacaatgctaagaccaagccaagagaggagcagtttaattccacataccgcgtggtgagcgtgctgaccgtgctgcatcaggattggctgaacggcaaggagtataagtgcaaggtgtccaataagggcctgcccagctctatcgagaagacaatcagcaaggctaagggacagcctagggagccacaggtgtacaccctgcccccttctcaggaggagatgacaaagaaccaggtgtccctgacctgtctggtgaagggcttctatccaagcgacatcgctgtggagtgggagtctaatggccagcccgagaacaattacaagaccacaccacccgtgctggactctgatggctccttctttctgtattctaggctgacagtggataagtcccggtggcaggagggcaacgtgtttagctgctctgtgatgcacgaggccctgcacaatcattatacccagaagtccctgagcctgtctctgggcaagtga

SEQ ID NO: 103 - protein, 215 aa, synthetic construct
  REGION 1..215: note = Light chain; note (original language) = 轻链
DIVMTQTPAIMSASPGEKVTMTCRASSSVSSTYLHWYQQKSGASPKLWIYTTSTLASGVPARFSGSGSGTSYSLTISSVEAEDAATYYCQQFSDSTWTFGGGTKLEIKRTVAAPSVFIFPPSDEQLKSGTASVVCLLNNFYPREAKVQWKVDNALQSGNSQESVTEQDSKDSTYSLSSTLTLSKADYEKHKVYACEVTHQGLSSPVTKSFNRGEC

SEQ ID NO: 104 - DNA, 648 bp, synthetic construct
  source 1..648: mol_type = other DNA
  gene 1..648: note = Nucleic acid encoding chimeric light chain; note (original language) = 轻链编码核酸
gacatcgtgatgacccagacacccgccatcatgtccgcctctcctggcgagaaggtgaccatgacatgcagggcctccagctccgtgtccagcacctacctgcactggtatcagcagaagagcggcgcttctccaaagctgtggatctacaccacatccacactggctagcggagtgccagctcggttctccggaagcggatctggcacctcctatagcctgacaatctcttccgtggaggccgaggacgccgctacctactattgtcagcagttctctgattccacctggacatttggcggcggcacaaagctggagatcaagcgtacggtggccgctcccagcgtgttcatctttcccccttctgacgagcagctgaagtctggcaccgcttccgtggtgtgcctgctgaacaatttctaccccagagaggccaaggtgcagtggaaggtggataacgctctgcagtccggcaatagccaggagtctgtgaccgagcaggactccaaggatagcacatattctctgtcttccaccctgacactgtctaaggccgactacgagaagcacaaggtgtatgcttgcgaggtgacccatcagggcctgagctctcctgtgacaaagtcctttaatcgcggcgagtgttga

SEQ ID NO: 105 - protein, 447 aa, synthetic construct
  REGION 1..447: note = Heavy chain; note (original language) = 重链
EVQLQQSGAEVARPGASVKLSCTVSGFNIEDDYIEWVKQRPEQGLEWIGRIDPANDKTKYAPKFQDKATITGDTSSNTAYLQLSSLTSEDTAVYYCTRPGLRRYYSMDYWGQGTSVTVSSASTKGPSVFPLAPCSRSTSESTAALGCLVKDYFPEPVTVSWNSGALTSGVHTFPAVLQSSGLYSLSSVVTVPSSSLGTKTYTCNVDHKPSNTKVDKRVESKYGPPCPPCPAPEFLGGPSVFLFPPKPKDTLMISRTPEVTCVVVDVSQEDPEVQFNWYVDGVEVHNAKTKPREEQFNSTYRVVSVLTVLHQDWLNGKEYKCKVSNKGLPSSIEKTISKAKGQPREPQVYTLPPSQEEMTKNQVSLTCLVKGFYPSDIAVEWESNGQPENNYKTTPPVLDSDGSFFLYSRLTVDKSRWQEGNVFSCSVMHEALHNHYTQKSLSLSLGK

SEQ ID NO: 106 - DNA, 1344 bp, synthetic construct
  source 1..1344: mol_type = other DNA
  gene 1..1344: note = Nucleic acid encoding chimeric heavy chain; note (original language) = 重链编码核酸
gaggtgcagctgcagcagtctggagctgaggtggctaggccaggagcttccgtgaagctgagctgcaccgtgtctggcttcaacatcgaggacgattacatcgagtgggtgaagcagagaccagagcagggactggagtggatcggaaggatcgaccccgccaacgataagacaaagtacgctcctaagtttcaggacaaggccaccatcacaggcgatacctccagcaatacagcttatctgcagctgtcttccctgacctccgaggacacagccgtgtactattgtaccagacccggcctgaggcggtactattccatggattattggggccagggcaccagcgtgacagtgagctctgcctctacaaagggcccttccgtgttcccactggctccctgctccagaagcacatctgagtccaccgccgctctgggctgtctggtgaaggactacttccctgagccagtgaccgtgtcctggaacagcggcgccctgacatctggcgtgcacacctttccagctgtgctgcagtccagcggcctgtactccctgtcttccgtggtgacagtgcccagctcttccctgggcaccaagacatatacctgcaacgtggaccataagccttccaataccaaggtggataagagggtggagagcaagtacggaccaccttgcccaccatgtccagctcctgagtttctgggaggaccatccgtgttcctgtttcctccaaagcctaaggacaccctgatgatcagccggacacctgaggtgacctgcgtggtggtggacgtgtctcaggaggatccagaggtgcagttcaactggtacgtggatggcgtggaggtgcacaatgctaagaccaagccaagagaggagcagtttaattccacataccgcgtggtgagcgtgctgaccgtgctgcatcaggattggctgaacggcaaggagtataagtgcaaggtgtccaataagggcctgcccagctctatcgagaagacaatcagcaaggctaagggacagcctagggagccacaggtgtacaccctgcccccttctcaggaggagatgacaaagaaccaggtgtccctgacctgtctggtgaagggcttctatccaagcgacatcgctgtggagtgggagtctaatggccagcccgagaacaattacaagaccacaccacccgtgctggactctgatggctccttctttctgtattctaggctgacagtggataagtcccggtggcaggagggcaacgtgtttagctgctctgtgatgcacgaggccctgcacaatcattatacccagaagtccctgagcctgtctctgggcaagtga

SEQ ID NO: 107 - protein, 214 aa, synthetic construct
  REGION 1..214: note = Light chain; note (original language) = 轻链
NIVLTQSPKSMSMSVGERVTLSCKASENVVSYVSWYQQKPEQSPKLLIYGASNRYTGVPDRFIGSGSSTDFTLIISSFQPEDLADYHCGQSYSYPLTFGAGTKLELKRTVAAPSVFIFPPSDEQLKSGTASVVCLLNNFYPREAKVQWKVDNALQSGNSQESVTEQDSKDSTYSLSSTLTLSKADYEKHKVYACEVTHQGLSSPVTKSFNRGEC

SEQ ID NO: 108 - DNA, 645 bp, synthetic construct
  source 1..645: mol_type = other DNA
  gene 1..645: note = Nucleic acid encoding chimeric light chain; note (original language) = 轻链编码核酸
aacatcgtgctgacccagtcccctaagagcatgtctatgtccgtgggcgagagggtgacactgtcttgcaaggcctccgagaacgtggtgtcctacgtgagctggtatcagcagaagcccgagcagagccctaagctgctgatctacggcgcttctaataggtataccggagtgccagaccggttcatcggatccggctccagcaccgatttcacactgatcatctcttcctttcagccagaggacctggccgattaccactgtggccagagctactcttatcccctgacctttggcgctggcacaaagctggagctgaagcgtacggtggccgctcccagcgtgttcatctttcccccttctgacgagcagctgaagtctggcaccgcttccgtggtgtgcctgctgaacaatttctaccccagagaggccaaggtgcagtggaaggtggataacgctctgcagtccggcaatagccaggagtctgtgaccgagcaggactccaaggatagcacatattctctgtcttccaccctgacactgtctaaggccgactacgagaagcacaaggtgtatgcttgcgaggtgacccatcagggcctgagctctcctgtgacaaagtcctttaatcgcggcgagtgttga

SEQ ID NO: 109 - protein, 444 aa, synthetic construct
  REGION 1..444: note = heavy chain; note (original language) = 重链
QVQLVQSGAEVKKPGSSVKVSCKASGYTFSRYWIEWVRQAPGQGLEWMGEFIPGSDTTNYAQKFQGRVTITADISTSTAYMELSSLRSEDTAVYYCARGGLRRMDYWGQGTLVTVSSASTKGPSVFPLAPCSRSTSESTAALGCLVKDYFPEPVTVSWNSGALTSGVHTFPAVLQSSGLYSLSSVVTVPSSSLGTKTYTCNVDHKPSNTKVDKRVESKYGPPCPPCPAPEFLGGPSVFLFPPKPKDTLMISRTPEVTCVVVDVSQEDPEVQFNWYVDGVEVHNAKTKPREEQFNSTYRVVSVLTVLHQDWLNGKEYKCKVSNKGLPSSIEKTISKAKGQPREPQVYTLPPSQEEMTKNQVSLTCLVKGFYPSDIAVEWESNGQPENNYKTTPPVLDSDGSFFLYSRLTVDKSRWQEGNVFSCSVMHEALHNHYTQKSLSLSLGK

SEQ ID NO: 110 - DNA, 1335 bp, synthetic construct
  source 1..1335: mol_type = other DNA
  gene 1..1335: note = nucleic acids encoding heavy chain; note (original language) = 重链编码核酸
caggtgcagctggtgcagagcggagctgaggtgaagaagccaggctccagcgtgaaggtgtcttgcaaggcttccggctacaccttctctagatattggatcgagtgggtgcgccaggctccaggacagggactggagtggatgggcgagttcatccctggctccgacaccacaaactacgctcagaagtttcagggcagggtgaccatcacagccgatatctccaccagcacagcttatatggagctgtcttccctgaggagcgaggacacagccgtgtactattgtgctagaggcggcctgaggcggatggattactggggccagggcaccctggtgacagtgagctctgcctctacaaagggcccttccgtgttcccactggctccctgctccagaagcacatctgagtccaccgccgctctgggctgtctggtgaaggactacttccctgagccagtgaccgtgtcctggaacagcggcgccctgacatctggcgtgcacacctttccagctgtgctgcagtccagcggcctgtactccctgtcttccgtggtgacagtgcccagctcttccctgggcaccaagacatatacctgcaacgtggaccataagccttccaataccaaggtggataagagggtggagagcaagtacggaccaccttgcccaccatgtccagctcctgagtttctgggaggaccatccgtgttcctgtttcctccaaagcctaaggacaccctgatgatcagccggacacctgaggtgacctgcgtggtggtggacgtgtctcaggaggatccagaggtgcagttcaactggtacgtggatggcgtggaggtgcacaatgctaagaccaagccaagagaggagcagtttaattccacataccgcgtggtgagcgtgctgaccgtgctgcatcaggattggctgaacggcaaggagtataagtgcaaggtgtccaataagggcctgcccagctctatcgagaagacaatcagcaaggctaagggacagcctagggagccacaggtgtacaccctgcccccttctcaggaggagatgacaaagaaccaggtgtccctgacctgtctggtgaagggcttctatccaagcgacatcgctgtggagtgggagtctaatggccagcccgagaacaattacaagaccacaccacccgtgctggactctgatggctccttctttctgtattctaggctgacagtggataagtcccggtggcaggagggcaacgtgtttagctgctctgtgatgcacgaggccctgcacaatcattatacccagaagtccctgagcctgtctctgggcaagtga

SEQ ID NO: 111 - protein, 215 aa, synthetic construct
  REGION 1..215: note = light chain; note (original language) = 轻链
DIQMTQSPSSLSASVGDRVTITCRASSSVSSTYLHWYQQKPGKAPKLLIYTTSTLASGVPSRFSGSGSGTDFTLTISSLQPEDFATYYCQQFSDSTWTFGQGTKLEIKRTVAAPSVFIFPPSDEQLKSGTASVVCLLNNFYPREAKVQWKVDNALQSGNSQESVTEQDSKDSTYSLSSTLTLSKADYEKHKVYACEVTHQGLSSPVTKSFNRGEC

SEQ ID NO: 112 - DNA, 648 bp, synthetic construct
  source 1..648: mol_type = other DNA
  gene 1..648: note = nucleic acid encoding light chain; note (original language) = 轻链编码核酸
gacatccagatgacacagagcccatccagcctgtccgccagcgtgggcgatagggtgaccatcacatgccgggcttcttccagcgtgtcttccacctacctgcactggtatcagcagaagcccggcaaggcccctaagctgctgatctacaccacaagcaccctggcttctggcgtgccatccaggttctctggctccggcagcggcacagactttaccctgacaatcagctctctgcagcccgaggacttcgccacctactattgtcagcagttctctgattccacctggacatttggccagggcacaaagctggagatcaagcgtacggtggccgctcccagcgtgttcatctttcccccttctgacgagcagctgaagtctggcaccgcttccgtggtgtgcctgctgaacaatttctaccccagagaggccaaggtgcagtggaaggtggataacgctctgcagtccggcaatagccaggagtctgtgaccgagcaggactccaaggatagcacatattctctgtcttccaccctgacactgtctaaggccgactacgagaagcacaaggtgtatgcttgcgaggtgacccatcagggcctgagctctcctgtgacaaagtcctttaatcgcggcgagtgttga

SEQ ID NO: 113 - protein, 444 aa, synthetic construct; identical to SEQ ID NO: 109
  REGION 1..444: note = heavy chain; note (original language) = 重链

SEQ ID NO: 114 - DNA, 1335 bp, synthetic construct; identical to SEQ ID NO: 110
  source 1..1335: mol_type = other DNA
  gene 1..1335: note = nucleic acid encoding heavy chain; note (original language) = 重链编码核酸

SEQ ID NO: 115 - protein, 215 aa, synthetic construct
  REGION 1..215: note = light chain; note (original language) = 轻链
DIQMTQSPSSLSASVGDRVTITCRASSSVSSTYLHWYQQKPGKAPKLLIYTTSTLASGVPSRFSGSGSGTDFTLTISSLQPEDFATYYCQQFSESTWTFGQGTKLEIKRTVAAPSVFIFPPSDEQLKSGTASVVCLLNNFYPREAKVQWKVDNALQSGNSQESVTEQDSKDSTYSLSSTLTLSKADYEKHKVYACEVTHQGLSSPVTKSFNRGEC

SEQ ID NO: 116 - DNA, 648 bp, synthetic construct
  source 1..648: mol_type = other DNA
  gene 1..648: note = nucleic acid encoding light chain; note (original language) = 轻链编码核酸
gacatccagatgacacagagcccatccagcctgtccgccagcgtgggcgatagggtgaccatcacatgccgggcttcttccagcgtgtcttccacctacctgcactggtatcagcagaagcccggcaaggcccctaagctgctgatctacaccacaagcaccctggcttctggcgtgccatccaggttctctggctccggcagcggcacagactttaccctgacaatcagctctctgcagcccgaggatttcgccacctactattgtcagcagttctctgagtccacctggacatttggccagggcacaaagctggagatcaagcgtacggtggccgctcccagcgtgttcatctttcccccttctgacgagcagctgaagtctggcaccgcttccgtggtgtgcctgctgaacaatttctaccccagagaggccaaggtgcagtggaaggtggataacgctctgcagtccggcaatagccaggagtctgtgaccgagcaggactccaaggatagcacatattctctgtcttccaccctgacactgtctaaggccgactacgagaagcacaaggtgtatgcttgcgaggtgacccatcagggcctgagctctcctgtgacaaagtcctttaatcgcggcgagtgttga

SEQ ID NO: 117 - protein, 444 aa, synthetic construct; identical to SEQ ID NO: 109
  REGION 1..444: note = heavy chain; note (original language) = 重链

SEQ ID NO: 118 - DNA, 1335 bp, synthetic construct; identical to SEQ ID NO: 110
  source 1..1335: mol_type = other DNA
  gene 1..1335: note = nucleic acid encoding heavy chain; note (original language) = 重链编码核酸

SEQ ID NO: 119 - protein, 215 aa, synthetic construct
  REGION 1..215: note = light chain; note (original language) = 轻链
DIQMTQSPSSLSASVGDRVTITCRASSSVSSTYLHWYQQKPGKAPKLLIYTTSTLASGVPSRFSGSGSGTSYTLTISSLQPEDFATYYCQQFSDSTWTFGQGTKLEIKRTVAAPSVFIFPPSDEQLKSGTASVVCLLNNFYPREAKVQWKVDNALQSGNSQESVTEQDSKDSTYSLSSTLTLSKADYEKHKVYACEVTHQGLSSPVTKSFNRGEC

SEQ ID NO: 120 - DNA, 648 bp, synthetic construct
  source 1..648: mol_type = other DNA
  gene 1..648: note = nucleic acid encoding light chain; note (original language) = 轻链编码核酸
gacatccagatgacacagagcccatccagcctgtccgccagcgtgggcgatagggtgaccatcacatgccgggcttcttccagcgtgtcttccacctacctgcactggtatcagcagaagcccggcaaggcccctaagctgctgatctacaccacaagcaccctggcttctggcgtgccatccaggttctctggctccggcagcggcacatcttataccctgacaatcagctctctgcagcccgaggactttgccacctactattgtcagcagttctctgattccacctggacatttggccagggcacaaagctggagatcaagcgtacggtggccgctcccagcgtgttcatctttcccccttctgacgagcagctgaagtctggcaccgcttccgtggtgtgcctgctgaacaatttctaccccagagaggccaaggtgcagtggaaggtggataacgctctgcagtccggcaatagccaggagtctgtgaccgagcaggactccaaggatagcacatattctctgtcttccaccctgacactgtctaaggccgactacgagaagcacaaggtgtatgcttgcgaggtgacccatcagggcctgagctctcctgtgacaaagtcctttaatcgcggcgagtgttga

SEQ ID NO: 121 - protein, 444 aa, synthetic construct; identical to SEQ ID NO: 109
  REGION 1..444: note = heavy chain; note (original language) = 重链

SEQ ID NO: 122 - DNA, 1335 bp, synthetic construct; identical to SEQ ID NO: 110
  source 1..1335: mol_type = other DNA
  gene 1..1335: note = nucleic acid encoding heavy chain; note (original language) = 重链编码核酸

SEQ ID NO: 123 - protein, 215 aa, synthetic construct
  REGION 1..215: note = light chain; note (original language) = 轻链
DIQMTQSPSSLSASVGDRVTITCRASSSVSSTYLHWYQQKPGKAPKLLIYTTSTLASGVPSRFSGSGSGTSYTLTISSLQPEDFATYYCQQFSESTWTFGQGTKLEIKRTVAAPSVFIFPPSDEQLKSGTASVVCLLNNFYPREAKVQWKVDNALQSGNSQESVTEQDSKDSTYSLSSTLTLSKADYEKHKVYACEVTHQGLSSPVTKSFNRGEC

SEQ ID NO: 124 - DNA, 648 bp, synthetic construct
  source 1..648: mol_type = other DNA
  gene 1..648: note = nucleic acids encoding light chain; note (original language) = 轻链编码核酸
gacatccagatgacacagagcccatccagcctgtccgccagcgtgggcgatagggtgaccatcacatgccgggcttcttccagcgtgtcttccacctacctgcactggtatcagcagaagcccggcaaggcccctaagctgctgatctacaccacaagcaccctggcttctggcgtgccatccaggttctctggctccggcagcggcacatcttataccctgacaatcagctctctgcagcccgaggactttgccacctactattgtcagcagttctctgagtccacctggacatttggccagggcacaaagctggagatcaagcgtacggtggccgctcccagcgtgttcatctttcccccttctgacgagcagctgaagtctggcaccgcttccgtggtgtgcctgctgaacaatttctaccccagagaggccaaggtgcagtggaaggtggataacgctctgcagtccggcaatagccaggagtctgtgaccgagcaggactccaaggatagcacatattctctgtcttccaccctgacactgtctaaggccgactacgagaagcacaaggtgtatgcttgcgaggtgacccatcagggcctgagctctcctgtgacaaagtcctttaatcgcggcgagtgttga

SEQ ID NO: 125 - protein, 444 aa, synthetic construct; identical to SEQ ID NO: 109
  REGION 1..444: note = heavy chain; note (original language) = 重链

SEQ ID NO: 126 - DNA, 1335 bp, synthetic construct; identical to SEQ ID NO: 110
  source 1..1335: mol_type = other DNA
  gene 1..1335: note = nucleic acid encoding heavy chain; note (original language) = 重链编码核酸

SEQ ID NO: 127 - protein, 215 aa, synthetic construct
  REGION 1..215: note = light chain; note (original language) = 轻链
DIQMTQSPSSLSASVGDRVTITCRASSSVSSTYLHWYQQKPGKAPKLWIYTTSTLASGVPSRFSGSGSGTSYTLTISSLQPEDFATYYCQQFSDSTWTFGQGTKLEIKRTVAAPSVFIFPPSDEQLKSGTASVVCLLNNFYPREAKVQWKVDNALQSGNSQESVTEQDSKDSTYSLSSTLTLSKADYEKHKVYACEVTHQGLSSPVTKSFNRGEC

SEQ ID NO: 128 - DNA, 648 bp, synthetic construct
  source 1..648: mol_type = other DNA
  gene 1..648: note = nucleic acid encoding light chain; note (original language) = 轻链编码核酸
gacatccagatgacacagagcccatccagcctgtccgccagcgtgggcgatagggtgaccatcacatgccgggcttcttccagcgtgtcttccacctacctgcactggtatcagcagaagcccggcaaggcccctaagctgtggatctacaccacaagcaccctggcttctggcgtgccatccaggttctctggctccggcagcggcacatcttataccctgacaatcagctctctgcagcccgaggactttgccacctactattgtcagcagttctctgattccacctggacatttggccagggcacaaagctggagatcaagcgtacggtggccgctcccagcgtgttcatctttcccccttctgacgagcagctgaagtctggcaccgcttccgtggtgtgcctgctgaacaatttctaccccagagaggccaaggtgcagtggaaggtggataacgctctgcagtccggcaatagccaggagtctgtgaccgagcaggactccaaggatagcacatattctctgtcttccaccctgacactgtctaaggccgactacgagaagcacaaggtgtatgcttgcgaggtgacccatcagggcctgagctctcctgtgacaaagtcctttaatcgcggcgagtgttga

SEQ ID NO: 129 - protein, 444 aa, synthetic construct; identical to SEQ ID NO: 109
  REGION 1..444: note = heavy chain; note (original language) = 重链

SEQ ID NO: 130 - DNA, 1335 bp, synthetic construct; identical to SEQ ID NO: 110
  source 1..1335: mol_type = other DNA
  gene 1..1335: note = nucleic acid encoding heavy chain; note (original language) = 重链编码核酸

SEQ ID NO: 131 - protein, 215 aa, synthetic construct
  REGION 1..215: note = light chain; note (original language) = 轻链
DIQMTQSPSSLSASVGDRVTITCRASSSVSSTYLHWYQQKPGKAPKLWIYTTSTLASGVPSRFSGSGSGTSYTLTISSLQPEDFATYYCQQFSESTWTFGQGTKLEIKRTVAAPSVFIFPPSDEQLKSGTASVVCLLNNFYPREAKVQWKVDNALQSGNSQESVTEQDSKDSTYSLSSTLTLSKADYEKHKVYACEVTHQGLSSPVTKSFNRGEC

SEQ ID NO: 132 - DNA, 648 bp, synthetic construct
  source 1..648: mol_type = other DNA
  gene 1..648: note = nucleic acid encoding light chain; note (original language) = 轻链编码核酸
gacatccagatgacacagagcccatccagcctgtccgccagcgtgggcgatagggtgaccatcacatgccgggcttcttccagcgtgtcttccacctacctgcactggtatcagcagaagcccggcaaggcccctaagctgtggatctacaccacaagcaccctggcttctggcgtgccatccaggttctctggctccggcagcggcacatcttataccctgacaatcagctctctgcagcccgaggactttgccacctactattgtcagcagttctctgagtccacctggacatttggccagggcacaaagctggagatcaagcgtacggtggccgctcccagcgtgttcatctttcccccttctgacgagcagctgaagtctggcaccgcttccgtggtgtgcctgctgaacaatttctaccccagagaggccaaggtgcagtggaaggtggataacgctctgcagtccggcaatagccaggagtctgtgaccgagcaggactccaaggatagcacatattctctgtcttccaccctgacactgtctaaggccgactacgagaagcacaaggtgtatgcttgcgaggtgacccatcagggcctgagctctcctgtgacaaagtcctttaatcgcggcgagtgttga

SEQ ID NO: 133 - protein, 444 aa, synthetic construct
  REGION 1..444: note = heavy chain; note (original language) = 重链
QVQLVQSGAEVKKPGSSVKVSCKASGYTFSRYWIEWVRQAPGQGLEWMGEFIPGSDTTNYAQKFQGRVTITAEISTNTAYMELSSLRSEDTAVYYCARGGLRRMDYWGQGTLVTVSSASTKGPSVFPLAPCSRSTSESTAALGCLVKDYFPEPVTVSWNSGALTSGVHTFPAVLQSSGLYSLSSVVTVPSSSLGTKTYTCNVDHKPSNTKVDKRVESKYGPPCPPCPAPEFLGGPSVFLFPPKPKDTLMISRTPEVTCVVVDVSQEDPEVQFNWYVDGVEVHNAKTKPREEQFNSTYRVVSVLTVLHQDWLNGKEYKCKVSNKGLPSSIEKTISKAKGQPREPQVYTLPPSQEEMTKNQVSLTCLVKGFYPSDIAVEWESNGQPENNYKTTPPVLDSDGSFFLYSRLTVDKSRWQEGNVFSCSVMHEALHNHYTQKSLSLSLGK

SEQ ID NO: 134 - DNA, 1335 bp, synthetic construct
  source 1..1335: mol_type = other DNA
  gene 1..1335: note = nucleic acid encoding heavy chain; note (original language) = 重链编码核酸
caggtgcagctggtgcagagcggagctgaggtgaagaagccaggctccagcgtgaaggtgtcctgcaaggctagcggctacaccttctctagatattggatcgagtgggtgcgccaggctccaggacagggactggagtggatgggcgagttcatccctggctccgacaccacaaactacgctcagaagtttcagggcagggtgaccatcacagccgagatctctaccaatacagcttatatggagctgtcttccctgaggtccgaggacacagccgtgtactattgtgctagaggcggcctgaggcggatggattactggggccagggcaccctggtgacagtgagctctgcctctacaaagggcccttccgtgttcccactggctccctgctccagaagcacatctgagtccaccgccgctctgggctgtctggtgaaggactacttccctgagccagtgaccgtgtcctggaacagcggcgccctgacatctggcgtgcacacctttccagctgtgctgcagtccagcggcctgtactccctgtcttccgtggtgacagtgcccagctcttccctgggcaccaagacatatacctgcaacgtggaccataagccttccaataccaaggtggataagagggtggagagcaagtacggaccaccttgcccaccatgtccagctcctgagtttctgggaggaccatccgtgttcctgtttcctccaaagcctaaggacaccctgatgatcagccggacacctgaggtgacctgcgtggtggtggacgtgtctcaggaggatccagaggtgcagttcaactggtacgtggatggcgtggaggtgcacaatgctaagaccaagccaagagaggagcagtttaattccacataccgcgtggtgagcgtgctgaccgtgctgcatcaggattggctgaacggcaaggagtataagtgcaaggtgtccaataagggcctgcccagctctatcgagaagacaatcagcaaggctaagggacagcctagggagccacaggtgtacaccctgcccccttctcaggaggagatgacaaagaaccaggtgtccctgacctgtctggtgaagggcttctatccaagcgacatcgctgtggagtgggagtctaatggccagcccgagaacaattacaagaccacaccacccgtgctggactctgatggctccttctttctgtattctaggctgacagtggataagtcccggtggcaggagggcaacgtgtttagctgctctgtgatgcacgaggccctgcacaatcattatacccagaagtccctgagcctgtctctgggcaagtga

SEQ ID NO: 135 - protein, 215 aa, synthetic construct; identical to SEQ ID NO: 111
  REGION 1..215: note = light chain; note (original language) = 轻链

SEQ ID NO: 136 - DNA, 648 bp, synthetic construct; identical to SEQ ID NO: 112
  source 1..648: mol_type = other DNA
  gene 1..648: note = nucleic acid encoding light chain; note (original language) = 轻链编码核酸

SEQ ID NO: 137 - protein, 444 aa, synthetic construct; identical to SEQ ID NO: 133
  REGION 1..444: note = heavy chain; note (original language) = 重链

SEQ ID NO: 138 - DNA, 1335 bp, synthetic construct; identical to SEQ ID NO: 134
  source 1..1335: mol_type = other DNA
  gene 1..1335: note = nucleic acid encoding heavy chain; note (original language) = 重链编码核酸

SEQ ID NO: 139 - protein, 215 aa, synthetic construct; identical to SEQ ID NO: 115
  REGION 1..215: note = light chain; note (original language) = 轻链

SEQ ID NO: 140 - DNA, 648 bp, synthetic construct; identical to SEQ ID NO: 116
  source 1..648: mol_type = other DNA
  gene 1..648: note = nucleic acid encoding light chain; note (original language) = 轻链编码核酸

SEQ ID NO: 141 - protein, 444 aa, synthetic construct; identical to SEQ ID NO: 133
  REGION 1..444: note = heavy chain; note (original language) = 重链

SEQ ID NO: 142 - DNA, 1335 bp, synthetic construct; identical to SEQ ID NO: 134
  source 1..1335: mol_type = other DNA
  gene 1..1335: note = nucleic acid encoding heavy chain; note (original language) = 重链编码核酸

SEQ ID NO: 143 - protein, 215 aa, synthetic construct; identical to SEQ ID NO: 119
  REGION 1..215: note = light chain; note (original language) = 轻链

SEQ ID NO: 144 - DNA, 648 bp, synthetic construct; identical to SEQ ID NO: 120
  source 1..648: mol_type = other DNA
  gene 1..648: note = nucleic acid encoding light chain; note (original language) = 轻链编码核酸

SEQ ID NO: 145 - protein, 444 aa, synthetic construct; identical to SEQ ID NO: 133
  REGION 1..444: note = heavy chain; note (original language) = 重链

SEQ ID NO: 146 - DNA, 1335 bp, synthetic construct; identical to SEQ ID NO: 134
  source 1..1335: mol_type = other DNA
  gene 1..1335: note = nucleic acid encoding heavy chain; note (original language) = 重链编码核酸

SEQ ID NO: 147 - protein, 215 aa, synthetic construct; identical to SEQ ID NO: 123
  REGION 1..215: note = light chain; note (original language) = 轻链

SEQ ID NO: 148 - DNA, 648 bp, synthetic construct; identical to SEQ ID NO: 124
  source 1..648: mol_type = other DNA
  gene 1..648: note = nucleic acid encoding light chain; note (original language) = 轻链编码核酸

SEQ ID NO: 149 - protein, 444 aa, synthetic construct; identical to SEQ ID NO: 133
  REGION 1..444: note = heavy chain; note (original language) = 重链

SEQ ID NO: 150 - DNA, 1335 bp, synthetic construct; identical to SEQ ID NO: 134
  source 1..1335: mol_type = other DNA
  gene 1..1335: note = nucleic acid encoding heavy chain; note (original language) = 重链编码核酸

SEQ ID NO: 151 - protein, 215 aa, synthetic construct; identical to SEQ ID NO: 127
  REGION 1..215: note = light chain; note (original language) = 轻链

SEQ ID NO: 152 - DNA, 648 bp, synthetic construct; identical to SEQ ID NO: 128
  source 1..648: mol_type = other DNA
  gene 1..648: note = nucleic acid encoding light chain; note (original language) = 轻链编码核酸

SEQ ID NO: 153 - protein, 444 aa, synthetic construct; identical to SEQ ID NO: 133
  REGION 1..444: note = heavy chain; note (original language) = 重链

SEQ ID NO: 154 - DNA, 1335 bp, synthetic construct; identical to SEQ ID NO: 134
  source 1..1335: mol_type = other DNA
  gene 1..1335: note = nucleic acid encoding heavy chain; note (original language) = 重链编码核酸

SEQ ID NO: 155 - protein, 215 aa, synthetic construct; identical to SEQ ID NO: 131
  REGION 1..215: note = light chain; note (original language) = 轻链

SEQ ID NO: 156 - DNA, 648 bp, synthetic construct; identical to SEQ ID NO: 132
  source 1..648: mol_type = other DNA
  gene 1..648: note = nucleic acid encoding light chain; note (original language) = 轻链编码核酸

SEQ ID NO: 157 - protein, 446 aa, synthetic construct
  REGION 1..446: note = heavy chain; note (original language) = 重链
QVQLVQSGAEVKKPGASVKVSCKASGYTFTNYGMNWVRQAPGQGLEWMGWINTNTGEPTYAQKLQGRVTMTLDTSTRTAYMELRSLRSDDTAVYYCARFSHLRGPMDYWGQGTLVTVSSASTKGPSVFPLAPCSRSTSESTAALGCLVKDYFPEPVTVSWNSGALTSGVHTFPAVLQSSGLYSLSSVVTVPSSSLGTKTYTCNVDHKPSNTKVDKRVESKYGPPCPPCPAPEFLGGPSVFLFPPKPKDTLMISRTPEVTCVVVDVSQEDPEVQFNWYVDGVEVHNAKTKPREEQFNSTYRVVSVLTVLHQDWLNGKEYKCKVSNKGLPSSIEKTISKAKGQPREPQVYTLPPSQEEMTKNQVSLTCLVKGFYPSDIAVEWESNGQPENNYKTTPPVLDSDGSFFLYSRLTVDKSRWQEGNVFSCSVMHEALHNHYTQKSLSLSLGK

SEQ ID NO: 158 - DNA, 1341 bp, synthetic construct
  source 1..1341: mol_type = other DNA
  gene 1..1341: note = nucleic acid encoding heavy chain; note (original language) = 重链编码核酸
caggtgcagctggtgcagtccggagctgaggtgaagaagccaggagctagcgtgaaggtgtcttgcaaggcctccggctacaccttcacaaactatggcatgaattgggtgaggcaggctccaggacagggactggagtggatgggctggatcaacaccaatacaggcgagcctacatacgcccagaagctgcagggcagggtgaccatgacactggacaccagcacaagaaccgcttatatggagctgaggtctctgcggtccgacgataccgccgtgtactattgtgctagattttctcacctgaggggaccaatggattactggggacagggcacactggtgaccgtgtccagcgcctctacaaagggcccttccgtgttcccactggctccctgctccagaagcacatctgagtccaccgccgctctgggctgtctggtgaaggactacttccctgagccagtgaccgtgtcctggaacagcggcgccctgacatctggcgtgcacacctttccagctgtgctgcagtccagcggcctgtactccctgtcttccgtggtgacagtgcccagctcttccctgggcaccaagacatatacctgcaacgtggaccataagccttccaataccaaggtggataagagggtggagagcaagtacggaccaccttgcccaccatgtccagctcctgagtttctgggaggaccatccgtgttcctgtttcctccaaagcctaaggacaccctgatgatcagccggacacctgaggtgacctgcgtggtggtggacgtgtctcaggaggatccagaggtgcagttcaactggtacgtggatggcgtggaggtgcacaatgctaagaccaagccaagagaggagcagtttaattccacataccgcgtggtgagcgtgctgaccgtgctgcatcaggattggctgaacggcaaggagtataagtgcaaggtgtccaataagggcctgcccagctctatcgagaagacaatcagcaaggctaagggacagcctagggagccacaggtgtacaccctgcccccttctcaggaggagatgacaaagaaccaggtgtccctgacctgtctggtgaagggcttctatccaagcgacatcgctgtggagtgggagtctaatggccagcccgagaacaattacaagaccacaccacccgtgctggactctgatggctccttctttctgtattctaggctgacagtggataagtcccggtggcaggagggcaacgtgtttagctgctctgtgatgcacgaggccctgcacaatcattatacccagaagtccctgagcctgtctctgggcaagtga

SEQ ID NO: 159 - protein, 219 aa, synthetic construct
  REGION 1..219: note = light chain; note (original language) = 轻链
DIQMTQSPSSLSASVGDRVTITCRSSQSLVHSNGYTYLHWYQQKPGKAPKLLIYKVSNRFSGVPSRFSGSGSGTDFTLTISSLQPEDFATYYCSQSTHVPPTFGQGTKLEIKRTVAAPSVFIFPPSDEQLKSGTASVVCLLNNFYPREAKVQWKVDNALQSGNSQESVTEQDSKDSTYSLSSTLTLSKADYEKHKVYACEVTHQGLSSPVTKSFNRGEC

SEQ ID NO: 160 - DNA, 660 bp, synthetic construct
  source 1..660: mol_type = other DNA
  gene 1..660: note = nucleic acid encoding light chain; note (original language) = 轻链编码核酸
gacatccagatgacacagtccccatccagcctgtccgccagcgtgggcgatagggtgaccatcacatgccggtcttcccagagcctggtgcactctaacggctacacctatctgcattggtaccagcagaagccaggcaaggctcccaagctgctgatctataaggtgtccaatagattcagcggcgtgccttctcgcttttctggctccggcagcggcacagacttcaccctgacaatcagctctctgcagccagaggattttgccacctactattgttctcagtccacccacgtgccccctacattcggccagggcaccaagctggagatcaagcgtacggtggccgctcccagcgtgttcatctttcccccttctgacgagcagctgaagtctggcaccgcttccgtggtgtgcctgctgaacaatttctaccccagagaggccaaggtgcagtggaaggtggataacgctctgcagtccggcaatagccaggagtctgtgaccgagcaggactccaaggatagcacatattctctgtcttccaccctgacactgtctaaggccgactacgagaagcacaaggtgtatgcttgcgaggtgacccatcagggcctgagctctcctgtgacaaagtcctttaatcgcggcgagtgttga

SEQ ID NO: 161 - protein, 446 aa, synthetic construct
  REGION 1..446: note = heavy chain; note (original language) = 重链
QVQLVQSGAEVKKPGASVKVSCKASGYTFTNYGMNWVRQAPGQGLKWMGWINTNTGEPTYAQELQGRVTMTLDTSTRTAYMELRSLRSDDTAVYYCTRFSHLRGPMDYWGQGTLVTVSSASTKGPSVFPLAPCSRSTSESTAALGCLVKDYFPEPVTVSWNSGALTSGVHTFPAVLQSSGLYSLSSVVTVPSSSLGTKTYTCNVDHKPSNTKVDKRVESKYGPPCPPCPAPEFLGGPSVFLFPPKPKDTLMISRTPEVTCVVVDVSQEDPEVQFNWYVDGVEVHNAKTKPREEQFNSTYRVVSVLTVLHQDWLNGKEYKCKVSNKGLPSSIEKTISKAKGQPREPQVYTLPPSQEEMTKNQVSLTCLVKGFYPSDIAVEWESNGQPENNYKTTPPVLDSDGSFFLYSRLTVDKSRWQEGNVFSCSVMHEALHNHYTQKSLSLSLGK

SEQ ID NO: 162 - DNA, 1341 bp, synthetic construct
  source 1..1341: mol_type = other DNA
  gene 1..1341: note = nucleic acid encoding heavy chain; note (original language) = 重链编码核酸
caggtgcagctggtgcagtccggagctgaggtgaagaagccaggagctagcgtgaaggtgtcttgcaaggcctccggctacaccttcacaaactatggcatgaattgggtgaggcaggctccaggacagggcctgaagtggatgggatggatcaacaccaatacaggcgagcctacatacgcccaggagctgcagggcagggtgaccatgacactggacaccagcacaagaaccgcctatatggagctgaggtctctgcggtccgacgatacagccgtgtactattgtaccagattttctcacctgaggggaccaatggattactggggacagggcacactggtgaccgtgtccagcgcctctacaaagggcccttccgtgttcccactggctccctgctccagaagcacatctgagtccaccgccgctctgggctgtctggtgaaggactacttccctgagccagtgaccgtgtcctggaacagcggcgccctgacatctggcgtgcacacctttccagctgtgctgcagtccagcggcctgtactccctgtcttccgtggtgacagtgcccagctcttccctgggcaccaagacatatacctgcaacgtggaccataagccttccaataccaaggtggataagagggtggagagcaagtacggaccaccttgcccaccatgtccagctcctgagtttctgggaggaccatccgtgttcctgtttcctccaaagcctaaggacaccctgatgatcagccggacacctgaggtgacctgcgtggtggtggacgtgtctcaggaggatccagaggtgcagttcaactggtacgtggatggcgtggaggtgcacaatgctaagaccaagccaagagaggagcagtttaattccacataccgcgtggtgagcgtgctgaccgtgctgcatcaggattggctgaacggcaaggagtataagtgcaaggtgtccaataagggcctgcccagctctatcgagaagacaatcagcaaggctaagggacagcctagggagccacaggtgtacaccctgcccccttctcaggaggagatgacaaagaaccaggtgtccctgacctgtctggtgaagggcttctatccaagcgacatcgctgtggagtgggagtctaatggccagcccgagaacaattacaagaccacaccacccgtgctggactctgatggctccttctttctgtattctaggctgacagtggataagtcccggtggcaggagggcaacgtgtttagctgctctgtgatgcacgaggccctgcacaatcattatacccagaagtccctgagcctgtctctgggcaagtga

SEQ ID NO: 163 - protein, 219 aa, synthetic construct; identical to SEQ ID NO: 159
  REGION 1..219: note = light chain; note (original language) = 轻链

SEQ ID NO: 164 - DNA, 660 bp, synthetic construct; identical to SEQ ID NO: 160
  source 1..660: mol_type = other DNA
  gene 1..660: note = nucleic acid encoding light chain; note (original language) = 轻链编码核酸

SEQ ID NO: 165 - protein, 446 aa, synthetic construct
  REGION 1..446: note = heavy chain; note (original language) = 重链
QVQLVQSGAEVKKPGASVKVSCKASGYTFTNYGMNWVRQAPGQGLKWMGWINTNTGEPTYAQELQGRVTMTLDTSTRTAYMELRSLRSDDTAVYYCARFSHLRGPMDYWGQGTLVTVSSASTKGPSVFPLAPCSRSTSESTAALGCLVKDYFPEPVTVSWNSGALTSGVHTFPAVLQSSGLYSLSSVVTVPSSSLGTKTYTCNVDHKPSNTKVDKRVESKYGPPCPPCPAPEFLGGPSVFLFPPKPKDTLMISRTPEVTCVVVDVSQEDPEVQFNWYVDGVEVHNAKTKPREEQFNSTYRVVSVLTVLHQDWLNGKEYKCKVSNKGLPSSIEKTISKAKGQPREPQVYTLPPSQEEMTKNQVSLTCLVKGFYPSDIAVEWESNGQPENNYKTTPPVLDSDGSFFLYSRLTVDKSRWQEGNVFSCSVMHEALHNHYTQKSLSLSLGK

SEQ ID NO: 166 - DNA, 1341 bp, synthetic construct
  source 1..1341: mol_type = other DNA
  gene 1..1341: note = nucleic acid encoding heavy chain; note (original language) = 重链编码核酸
caggtgcagctggtgcagtccggagctgaggtgaagaagccaggagctagcgtgaaggtgtcttgcaaggcctccggctacaccttcacaaactatggcatgaattgggtgaggcaggctccaggacagggcctgaagtggatgggatggatcaacaccaatacaggcgagcctacatacgcccaggagctgcagggcagggtgaccatgacactggacaccagcacaagaaccgcttatatggagctgaggtctctgcggtccgacgataccgccgtgtactattgtgctagattttctcacctgaggggaccaatggattactggggacagggcacactggtgaccgtgtccagcgcctctacaaagggcccttccgtgttcccactggctccctgctccagaagcacatctgagtccaccgccgctctgggctgtctggtgaaggactacttccctgagccagtgaccgtgtcctggaacagcggcgccctgacatctggcgtgcacacctttccagctgtgctgcagtccagcggcctgtactccctgtcttccgtggtgacagtgcccagctcttccctgggcaccaagacatatacctgcaacgtggaccataagccttccaataccaaggtggataagagggtggagagcaagtacggaccaccttgcccaccatgtccagctcctgagtttctgggaggaccatccgtgttcctgtttcctccaaagcctaaggacaccctgatgatcagccggacacctgaggtgacctgcgtggtggtggacgtgtctcaggaggatccagaggtgcagttcaactggtacgtggatggcgtggaggtgcacaatgctaagaccaagccaagagaggagcagtttaattccacataccgcgtggtgagcgtgctgaccgtgctgcatcaggattggctgaacggcaaggagtataagtgcaaggtgtccaataagggcctgcccagctctatcgagaagacaatcagcaaggctaagggacagcctagggagccacaggtgtacaccctgcccccttctcaggaggagatgacaaagaaccaggtgtccctgacctgtctggtgaagggcttctatccaagcgacatcgctgtggagtgggagtctaatggccagcccgagaacaattacaagaccacaccacccgtgctggactctgatggctccttctttctgtattctaggctgacagtggataagtcccggtggcaggagggcaacgtgtttagctgctctgtgatgcacgaggccctgcacaatcattatacccagaagtccctgagcctgtctctgggcaagtga

SEQ ID NO: 167 - protein, 219 aa, synthetic construct; identical to SEQ ID NO: 159
  REGION 1..219: note = light chain; note (original language) = 轻链

SEQ ID NO: 168 - DNA, 660 bp, synthetic construct; identical to SEQ ID NO: 160
  source 1..660: mol_type = other DNA
  gene 1..660: note = nucleic acid encoding light chain; note (original language) = 轻链编码核酸

SEQ ID NO: 169 - protein, 446 aa, synthetic construct; identical to SEQ ID NO: 165
  REGION 1..446: note = heavy chain; note (original language) = 重链

SEQ ID NO: 170 - DNA, 1341 bp, synthetic construct; identical to SEQ ID NO: 166
  source 1..1341: mol_type = other DNA
  gene 1..1341: note = nucleic acid encoding heavy chain; note (original language) = 重链编码核酸

SEQ ID NO: 171 - protein, 219 aa, synthetic construct
  REGION 1..219: note = light chain; note (original language) = 轻链
DAQMTQSPSSLSASVGDRVTITCRSSQSLVHSNGYTYLHWYQQKPGKAPKLLIYKVSNRFSGVPSRFSGSGSGTDFTLTISSLQPEDFATYYCSQSTHVPPTFGQGTKLEIKRTVAAPSVFIFPPSDEQLKSGTASVVCLLNNFYPREAKVQWKVDNALQSGNSQESVTEQDSKDSTYSLSSTLTLSKADYEKHKVYACEVTHQGLSSPVTKSFNRGEC

SEQ ID NO: 172 - DNA, 660 bp, synthetic construct
  source 1..660: mol_type = other DNA
  gene 1..660: note = nucleic acid encoding light chain; note (original language) = 轻链编码核酸
gacgcccagatgacacagtccccatccagcctgtccgctagcgtgggcgatagggtgaccatcacatgccggtcttcccagagcctggtgcactctaacggctacacctatctgcattggtaccagcagaagccaggcaaggcccccaagctgctgatctataaggtgtccaatagattcagcggcgtgccttctcgcttttctggctccggcagcggcacagacttcaccctgacaatcagctctctgcagccagaggattttgctacctactattgttctcagtccacccacgtgccccctacattcggccagggcaccaagctggagatcaagcgtacggtggccgctcccagcgtgttcatctttcccccttctgacgagcagctgaagtctggcaccgcttccgtggtgtgcctgctgaacaatttctaccccagagaggccaaggtgcagtggaaggtggataacgctctgcagtccggcaatagccaggagtctgtgaccgagcaggactccaaggatagcacatattctctgtcttccaccctgacactgtctaaggccgactacgagaagcacaaggtgtatgcttgcgaggtgacccatcagggcctgagctctcctgtgacaaagtcctttaatcgcggcgagtgttga

SEQ ID NO: 173 - protein, 446 aa, synthetic construct; identical to SEQ ID NO: 157
  REGION 1..446: note = heavy chain; note (original language) = 重链

SEQ ID NO: 174 - DNA, 1341 bp, synthetic construct; identical to SEQ ID NO: 158
  source 1..1341: mol_type = other DNA
  gene 1..1341: note = nucleic acid encoding heavy chain; note (original language) = 重链编码核酸

SEQ ID NO: 175 - protein, 219 aa, synthetic construct; identical to SEQ ID NO: 171
  REGION 1..219: note = light chain; note (original language) = 轻链

SEQ ID NO: 176 - DNA, 660 bp, synthetic construct; identical to SEQ ID NO: 172
  source 1..660: mol_type = other DNA
  gene 1..660: note = nucleic acid encoding light chain; note (original language) = 轻链编码核酸

SEQ ID NO: 177 - protein, 446 aa, synthetic construct; identical to SEQ ID NO: 161
  REGION 1..446: note = heavy chain; note (original language) = 重链

SEQ ID NO: 178 - DNA, 1341 bp, synthetic construct; identical to SEQ ID NO: 162
  source 1..1341: mol_type = other DNA
  gene 1..1341: note = nucleic acid encoding heavy chain; note (original language) = 重链编码核酸

SEQ ID NO: 179 - protein, 219 aa, synthetic construct; identical to SEQ ID NO: 171
  REGION 1..219: note = light chain; note (original language) = 轻链

SEQ ID NO: 180 - DNA, 660 bp, synthetic construct; identical to SEQ ID NO: 172
  source 1..660: mol_type = other DNA
  gene 1..660: note = nucleic acid encoding light chain; note (original language) = 轻链编码核酸

SEQ ID NO: 181 - protein, 447 aa, synthetic construct
  REGION 1..447: note = heavy chain; note (original language) = 重链
QVQLVQSGAEVKKPGASVKVSCKVSGFNIEDDYIEWVRQAPGQGLEWMGRIDPANDKTKYAQKFQGRVTMTGDTSTNTVYMELSSLRSEDTAVYYCARPGLRRYYSMDYWGQGTLVTVSSASTKGPSVFPLAPCSRSTSESTAALGCLVKDYFPEPVTVSWNSGALTSGVHTFPAVLQSSGLYSLSSVVTVPSSSLGTKTYTCNVDHKPSNTKVDKRVESKYGPPCPPCPAPEFLGGPSVFLFPPKPKDTLMISRTPEVTCVVVDVSQEDPEVQFNWYVDGVEVHNAKTKPREEQFNSTYRVVSVLTVLHQDWLNGKEYKCKVSNKGLPSSIEKTISKAKGQPREPQVYTLPPSQEEMTKNQVSLTCLVKGFYPSDIAVEWESNGQPENNYKTTPPVLDSDGSFFLYSRLTVDKSRWQEGNVFSCSVMHEALHNHYTQKSLSLSLGK

SEQ ID NO: 182 - DNA, 1344 bp, synthetic construct
  source 1..1344: mol_type = other DNA
  gene 1..1344: note = nucleic acid encoding heavy chain; note (original language) = 重链编码核酸
caggtgcagctggtgcagtccggagctgaggtgaagaagccaggagctagcgtgaaggtgtcttgcaaggtgtccggcttcaacatcgaggacgattacatcgagtgggtgaggcaggctccaggacagggactggagtggatgggaaggatcgaccctgccaacgataagacaaagtacgctcagaagtttcagggcagagtgaccatgacaggcgacaccagcacaaataccgtgtatatggagctgtccagcctgcgctctgaggataccgccgtgtactattgtgctaggcccggcctgagacgctactattccatggactattggggccagggcacactggtgaccgtgtcttccgcctctacaaagggcccttccgtgttcccactggctccctgctccagaagcacatctgagtccaccgccgctctgggctgtctggtgaaggactacttccctgagccagtgaccgtgtcctggaacagcggcgccctgacatctggcgtgcacacctttccagctgtgctgcagtccagcggcctgtactccctgtcttccgtggtgacagtgcccagctcttccctgggcaccaagacatatacctgcaacgtggaccataagccttccaataccaaggtggataagagggtggagagcaagtacggaccaccttgcccaccatgtccagctcctgagtttctgggaggaccatccgtgttcctgtttcctccaaagcctaaggacaccctgatgatcagccggacacctgaggtgacctgcgtggtggtggacgtgtctcaggaggatccagaggtgcagttcaactggtacgtggatggcgtggaggtgcacaatgctaagaccaagccaagagaggagcagtttaattccacataccgcgtggtgagcgtgctgaccgtgctgcatcaggattggctgaacggcaaggagtataagtgcaaggtgtccaataagggcctgcccagctctatcgagaagacaatcagcaaggctaagggacagcctagggagccacaggtgtacaccctgcccccttctcaggaggagatgacaaagaaccaggtgtccctgacctgtctggtgaagggcttctatccaagcgacatcgctgtggagtgggagtctaatggccagcccgagaacaattacaagaccacaccacccgtgctggactctgatggctccttctttctgtattctaggctgacagtggataagtcccggtggcaggagggcaacgtgtttagctgctctgtgatgcacgaggccctgcacaatcattatacccagaagtccctgagcctgtctctgggcaagtga

SEQ ID NO: 183 - protein, 214 aa, synthetic construct
  REGION 1..214: note = light chain; note (original language) = 轻链
DIQMTQSPSSLSASVGDRVTITCKASENVVSYVSWYQQKPGKAPKLLIYGASNRYTGVPSRFIGSGSSTDFTLTISSLQPEDFATYYCGQSYSYPLTFGQGTKLEIKRTVAAPSVFIFPPSDEQLKSGTASVVCLLNNFYPREAKVQWKVDNALQSGNSQESVTEQDSKDSTYSLSSTLTLSKADYEKHKVYACEVTHQGLSSPVTKSFNRGEC

SEQ ID NO: 184 - DNA, 645 bp, synthetic construct
  source 1..645: mol_type = other DNA
  gene 1..645: note = nucleic acid encoding light chain; note (original language) = 轻链编码核酸
gacatccagatgacccagagcccttccagcctgtccgccagcgtgggcgatagggtgaccatcacatgcaaggcttctgagaacgtggtgtcctacgtgagctggtatcagcagaagcccggcaaggcccctaagctgctgatctacggcgcttctaataggtataccggagtgccatcccggttcatcggatccggctcttccacagactttaccctgacaatcagctctctgcagccagaggatttcgccacatactattgtggccagagctactcttatcccctgacctttggccagggcacaaagctggagatcaagcgtacggtggccgctcccagcgtgttcatctttcccccttctgacgagcagctgaagtctggcaccgcttccgtggtgtgcctgctgaacaatttctaccccagagaggccaaggtgcagtggaaggtggataacgctctgcagtccggcaatagccaggagtctgtgaccgagcaggactccaaggatagcacatattctctgtcttccaccctgacactgtctaaggccgactacgagaagcacaaggtgtatgcttgcgaggtgacccatcagggcctgagctctcctgtgacaaagtcctttaatcgcggcgagtgttga

SEQ ID NO: 185 - protein, 447 aa, synthetic construct
  REGION 1..447: note = heavy chain; note (original language) = 重链
QVQLVQSGAEVKKPGASVKVSCKVSGFNIEDDYIEWVRQAPGQGLEWMGRIDPANDKTKYAQKFQGRVTMTGDTSTNTVYMELSSLRSEDTAVYYCTRPGLRRYYSMDYWGQGTLVTVSSASTKGPSVFPLAPCSRSTSESTAALGCLVKDYFPEPVTVSWNSGALTSGVHTFPAVLQSSGLYSLSSVVTVPSSSLGTKTYTCNVDHKPSNTKVDKRVESKYGPPCPPCPAPEFLGGPSVFLFPPKPKDTLMISRTPEVTCVVVDVSQEDPEVQFNWYVDGVEVHNAKTKPREEQFNSTYRVVSVLTVLHQDWLNGKEYKCKVSNKGLPSSIEKTISKAKGQPREPQVYTLPPSQEEMTKNQVSLTCLVKGFYPSDIAVEWESNGQPENNYKTTPPVLDSDGSFFLYSRLTVDKSRWQEGNVFSCSVMHEALHNHYTQKSLSLSLGK

SEQ ID NO: 186 - DNA, 1344 bp, synthetic construct
  source 1..1344: mol_type = other DNA
  gene 1..1344: note = nucleic acid encoding heavy chain; note (original language) = 重链编码核酸
caggtgcagctggtgcagtccggagctgaggtgaagaagccaggagctagcgtgaaggtgtcttgcaaggtgtccggcttcaacatcgaggacgattacatcgagtgggtgaggcaggctccaggacagggactggagtggatgggaaggatcgaccctgccaacgataagacaaagtacgctcagaagtttcagggcagagtgaccatgacaggcgacaccagcacaaataccgtgtatatggagctgtccagcctgcgctctgaggatacagccgtgtactattgtaccaggcccggcctgagacgctactattccatggactattggggccagggcacactggtgaccgtgtcttccgcctctacaaagggcccttccgtgttcccactggctccctgctccagaagcacatctgagtccaccgccgctctgggctgtctggtgaaggactacttccctgagccagtgaccgtgtcctggaacagcggcgccctgacatctggcgtgcacacctttccagctgtgctgcagtccagcggcctgtactccctgtcttccgtggtgacagtgcccagctcttccctgggcaccaagacatatacctgcaacgtggaccataagccttccaataccaaggtggataagagggtggagagcaagtacggaccaccttgcccaccatgtccagctcctgagtttctgggaggaccatccgtgttcctgtttcctccaaagcctaaggacaccctgatgatcagccggacacctgaggtgacctgcgtggtggtggacgtgtctcaggaggatccagaggtgcagttcaactggtacgtggatggcgtggaggtgcacaatgctaagaccaagccaagagaggagcagtttaattccacataccgcgtggtgagcgtgctgaccgtgctgcatcaggattggctgaacggcaaggagtataagtgcaaggtgtccaataagggcctgcccagctctatcgagaagacaatcagcaaggctaagggacagcctagggagccacaggtgtacaccctgcccccttctcaggaggagatgacaaagaaccaggtgtccctgacctgtctggtgaagggcttctatccaagcgacatcgctgtggagtgggagtctaatggccagcccgagaacaattacaagaccacaccacccgtgctggactctgatggctccttctttctgtattctaggctgacagtggataagtcccggtggcaggagggcaacgtgtttagctgctctgtgatgcacgaggccctgcacaatcattatacccagaagtccctgagcctgtctctgggcaagtga

SEQ ID NO: 187 - protein, 214 aa, synthetic construct; identical to SEQ ID NO: 183
  REGION 1..214: note = light chain; note (original language) = 轻链

SEQ ID NO: 188 - DNA, 645 bp, synthetic construct; identical to SEQ ID NO: 184
  source 1..645: mol_type = other DNA
  gene 1..645: note = nucleic acid encoding light chain; note (original language) = 轻链编码核酸

SEQ ID NO: 189 - DNA, 348 bp, Mus musculus
  source 1..348: mol_type = other DNA
caggtgcagctgaaggagtctggaccaggactggtggctccatctcagtccctgagcatcacctgcacagtgtccggcttcagcctgaccaactacggagtgcactgggtgaggcagccacctggcaagggactggagtggctgggcatcatctgggctggcggctccacaaactataattctgccctgatgtcccggctgtctatctccaaggacaacagcaagtctcaggtgtttctgaagatgaatagcctgcagaccgacgatacagccatgtactattgtgctagggacgattacgccagcatggattattggggccagggcacctctgtgacagtgtccagc

SEQ ID NO: 190 - DNA, 336 bp, Mus musculus
  source 1..336: mol_type = other DNA
gacgccttcatgacccagacaccactgtccctgcctgtgagcctgggcgatcaggcttctatctcctgcagatccagccagtctctggtgcactccaacggcaatacatacctgcattggtatctgcagaagccaggccagtcccccaagctgctgatctacaaggtgagcaacaggttctctggcgtgcctgaccggtttagcggctctggctccggcaccgatttcacactgaagatctccagggtggaggctgaggacctgggcgtgtacttttgtagccagtctacccacgtgccatatacactgggcggcggcaccaagctggagatcaag

SEQ ID NO: 191 - DNA, 357 bp, Mus musculus
  source 1..357: mol_type = other DNA
gaggtgcagctgcagcagtctggccccgagctgaagaagcctggcgagaccgtgaagatctcttgcaaggcctccggctacaccttcacaaactatggcatgaattgggtgaagcaggtgccaggcaagggcctgaagtggatgggctggatcaacaccaatacaggcgagcccacatacgccgaggagttcaagggcagattcgcttttagcctggagacctctgcccgcacagcttttctgcagatcaacaatctgaagaacgaggacaccgccacatacttctgtaccaggttttcccacctgcggggccccatggattattggggccagggcgctagcgtgacagtgtccagc

SEQ ID NO: 192 - DNA, 336 bp, Mus musculus
  source 1..336: mol_type = other DNA
gacgccgtgatgacccagacaccactgtccctgcccgtgagcctgggcgatcaggcttctatctcctgcagatccagccagtctctggtgcactccaacggctacacatatctgcattggtacctgcagaagcctggccagtccccaaagctgctgatctataaggtgagcaataggttctctggagtgccagaccggtttagcggatctggatccggcaccgatttcacactgaagatctccaggctggaggctgaggacctgggcgtgtacttctgtagccagtctacccacgtgccccctacatttggcggcggcaccaagctggagatcaag

SEQ ID NO: 193 - DNA, 336 bp, Mus musculus
  source 1..336: mol_type = other DNA
gaagtgatgctggtggagagcggaggaggactggtgcagccaggaggcagcctgaagctgtcttgcgccgcttccggcttcacctttagcaactactatatgtcttgggtgagacagacacccgagaagcgcctggagtgggtggcttacatctccagcggaggaggatccacctactatcctgacagcgtgaagggcaggttcaccatctctcgggataacgccaagaatacactgtacctgcagatgtcttccctgaagtccgaggacacagctatgtactattgtgcctggtttgcttattggggccagggcaccctggtgacagtgtctgct

SEQ ID NO: 194 - DNA, 336 bp, Mus musculus
  source 1..336: mol_type = other DNA
gacgccgtggtgacccagacaccactgaccctgtccgtgacaatcggccagcccgcttctatctcctgcaagtccagccagtccctgctggacagcgatggcaagacatacctgaactggctgctgcagaggccaggacagagccctaagcggctgatctatctggtgtctaagctggactccggcgtgcctgatagattcaccggcagcggctctggcaccgactttacactgaagatctctcgcgtggaggccgaggatctgggcgtgtactattgttggcagggcacccacttcccactgacatttggcgctggcaccaagctggagctgaag

SEQ ID NO: 195 - DNA, 351 bp, Mus musculus
  source 1..351: mol_type = other DNA
gaggtgcagctgcagcagtctgtggccgagctgatgaagccaggcgcttccgtgaagatctactgcaaggccaccggctacacattcagcagatattggatcgagtgggtgaagcagaggccaggacacggactggagtggatcggcgagttcatccctggctctgacaccacaaacttcaatgagaagtttaagggcaaggccacctttacagctgagatctccagcaacaccgcttatatgcagctgtcttccctgacatccgaggacagcgccgtgtacttttgtgctaggggcggcctgaggcggatggattattggggccagggcacctccgtgacagtgagctct

SEQ ID NO: 196 - DNA, 324 bp, Mus musculus
  source 1..324: mol_type = other DNA
gacatcgtgatgacccagacacccgccatcatgtccgcctctcctggcgagaaggtgaccatgacatgcagggcctccagctccgtgtccagcacctacctgcactggtatcagcagaagagcggcgcttctccaaagctgtggatctacaccacatccacactggctagcggagtgccagctcggttctccggaagcggatctggcacctcctatagcctgacaatctcttccgtggaggccgaggacgccgctacctactattgtcagcagttctctgattccacctggacatttggcggcggcacaaagctggagatcaag

SEQ ID NO: 197 - DNA, 360 bp, Mus musculus
  source 1..360: mol_type = other DNA
gaggtgcagctgcagcagtctggagctgaggtggctaggccaggagcttccgtgaagctgagctgcaccgtgtctggcttcaacatcgaggacgattacatcgagtgggtgaagcagagaccagagcagggactggagtggatcggaaggatcgaccccgccaacgataagacaaagtacgctcctaagtttcaggacaaggccaccatcacaggcgatacctccagcaatacagcttatctgcagctgtcttccctgacctccgaggacacagccgtgtactattgtaccagacccggcctgaggcggtactattccatggattattggggccagggcaccagcgtgacagtgagctct

SEQ ID NO: 198 - DNA, 321 bp, Mus musculus
  source 1..321: mol_type = other DNA
aacatcgtgctgacccagtcccctaagagcatgtctatgtccgtgggcgagagggtgacactgtcttgcaaggcctccgagaacgtggtgtcctacgtgagctggtatcagcagaagcccgagcagagccctaagctgctgatctacggcgcttctaataggtataccggagtgccagaccggttcatcggatccggctccagcaccgatttcacactgatcatctcttcctttcagccagaggacctggccgattaccactgtggccagagctactcttatcccctgacctttggcgctggcacaaagctggagctgaag